European Patent Specification EP 2 758 075 B1, published May 3, 2023. Title: INFLUENZA VIRUS VACCINES AND USES THEREOF. Applicant: Mount Sinai School of Medicine. The sequence listing filed with the application follows.

SEQUENCE LISTING (582 sequences)

SEQ ID NO: 1 - protein, 565 aa, Influenza virus A
  influenza virus A hemagglutinin subtype H1
MKANLLVLLCALAAADADTICIGYHANNSTDTVDTVLEKNVTVTHSVNLLEDSHNGKLCRLKGIAPLQLGKCNIAGWLLGNPECDPLLPVRSWSYIVETPNSENGICYPGDFIDYEELREQLSSVSSFERFEIFPKESSWPNHNTNGVTAACSHEGKSSFYRNLLWLTEKEGSYPKLKNSYVNKKGKEVLVLWGIHHPPNSKEQQNLYQNENAYVSVVTSNYNRRFTPEIAERPKVRDQAGRMNYYWTLLKPGDTIIFEANGNLIAPMYAFALSRGFGSGIITSNASMHECNTKCQTPLGAINSSLPYQNIHPVTIGECPKYVRSAKLRMVTGLRNNPSIQSRGLFGAIAGFIEGGWTGMIDGWYGYHHQNEQGSGYAADQKSTQNAINGITNKVNTVIEKMNIQFTAVGKEFNKLEKRMENLNKKVDDGFLDIWTYNAELLVLLENERTLDFHDSNVKNLYEKVKSQLKNNAKEIGNGCFEFYHKCDNECMESVRNGTYDYPKYSEESKLNREKVDGVKLESMGIYQILAIYSTVASSLVLLVSLGAISFWMCSNGSLQCRICI

SEQ ID NO: 2 - protein, 562 aa, Influenza virus A
  influenza virus A hemagglutinin subtype H2
MAIIYLILLFTAVRGDQICIGYHSNNSTEKVDTILERNVTVTHAQNILEKTHNGKLCKLNGIPPLELGDCSIAGWLLGNPECDRLLTVPEWSYIMEKENPRNGLCYPGSFNDYEELKHLLSSVTHFEKVKILPKDRWTQHTTTGGSRACAVSGNPSFFRNMVWLTKKGSNYPIAKGSYNNTSGEQMLIIWGVHHPNDETEQRTLYQNVGTYVSIGTSTLNKRSIPVIATRPKVNGQGGRMEFSWTILDIWDTINFESTGNLIAPEYGFRISKRGSSGIMKTEGTLENCETKCQTPLGAINTTLPFHNVHPLTIGECPKYVKSERLVLATGLRNVPQIESRGLFGAIAGFIEGGWQGMIDGWYGYHHSNDQGSGYAADKESTQKAIDGITNRVNSVIEKMNTQFEAVGKEFSNLEKRLENLNKKMEDGFLDVWTYNAELLVLMENERTLDFHDSNVKNLYDRVRMQLRDNAKELGNGCFEFYHKCDDECMNSVKNGTYDYPKYEEESKLNRNEIKGVKLSNMGVYQILAIYATVAGSLSLAIMIAGISLWMCSNGSLQCRICI

SEQ ID NO: 3 - protein, 566 aa, Influenza virus A
  influenza virus A hemagglutinin subtype H3
MKTIIALSYIFCLALGQDLPGNDNSTATLCLGHHAVPNGTLVKTITDDQIEVTNATELVQSSSTGKICNNPHRILDGIDCTLIDALLGDPHCDVFQNETWDLFVERSKAFSNCYPYDVPDYASLRSLVASSGTLEFITEGFTWTGVTQNGGSNACKRGPGNGFFSRLNWLTKSGSTYPVLNVTMPNNDNFDKLYIWGVHHPSTNQEQTSLYVQESGRVTVSTRRSQQSIIPNIGSRPWVRGQSSRISIYWTIVKPGDVLVINSNGNLIAPRGYFKMRTGKSSIMSSDAPIDTCISECITPNGSIPNDKPFQNVNKITYGACPKYVKQNTLKLATGMRNVPEKQTRGLFGAIAGFIENGWEGMIDGWYGFRHQNSEGTGQAADLKSTQAAIDQINGKLNRVIEKTNEKFHQIEKEFSEVEGRIQDLEKYVEDTKIDLWSYNAELLVALENQHTIDLTDSEMNKLFEKTRRQLRENAEDMGNGCFKIYHKCDNACIESIRNGTYDHDVYRDEALNNRFQIKGVELKSGYKDWILWISFAISCFLLCVVLLGFIMWACQRGNIRCNICI

SEQ ID NO: 4 - protein, 564 aa, Influenza virus A
  influenza virus A hemagglutinin subtype H4
MLSIVILFLLIAENSSQNYTGNPVICMGHHAVANGTMVKTLADDQVEVVTAQELVESQNLPELCPSPLRLVDGQTCDIINGALGSPGCDHLNGAEWDVFIERPNAVDTCYPFDVPEYQSLRSILANNGKFEFIAEEFQWNTVKQNGKSGACKRANVDDFFNRLNWLVKSDGNAYPLQNLTKINNGDYARLYIWGVHHPSTSTEQTNLYKNNPGRVTVSTKTSQTSVVPDIGSRPLVRGQSGRVSFYWTIVEPGDLIVFNTIGNLIAPRGHYKLNNQKKSTILNTAIPIGSCVSKCHTDKGSLSTTKPFQNISRIAVGDCPRYVKQGSLKLATGMRNIPEKASRGLFGAIAGFIENGWQGLIDGWYGFRHQNAEGTGTAADLKSTQAAIDQINGKLNRLIEKTNDKYHQIEKEFEQVEGRIQDLENYVEDTKIDLWSYNAELLVALENQHTIDVTDSEMNKLFERVRRQLRENAEDKGNGCFEIFHKCDNNCIESIRNGTYDHDIYRDEAINNRFQIQGVKLTQGYKDIILWISFSISCFLLVALLLAFILWACQNGNIRCQICI

SEQ ID NO: 5 - protein, 564 aa, Influenza virus A
  influenza virus A hemagglutinin subtype H5
MERIVLLLAIVSLVKSDQICIGYHANKSTKQVDTIMEKNVTVTHAQDILERTHNGKLCSLNGVKPLILRDCSVAGWLLGNPMCDEFLNLPEWLYIVEKDNPINSLCYPGDFNDYEELKYLLSSTNHFEKIRIIPRSSWSNHDASSGVSSACPYIGRSSFLRNVVWLIKKNNTYPTIKRSYNNTNQEDLLILWGIHHPNDAAEQTKLYQNPTTYVSVGTSTLNQRSIPEIATRPKVNGQSGRMEFFWTILKPNDAINFESNGNFIAPRYAYKIVKKGDSAIMKSGLAYGNCDTKCQTPVGEINSSMPFHNIHPHTIGECPKYVKSDRLVLATGLRNVPQRKKRGLFGAIAGFIEGGWQGMVDGWYGYHHSNEQGSGYAADKESTQKAIDGITNKVNSIIDKMNTRFEAVGKEFNNLERRVENLNKKMEDGFLDVWTYNVELLVLMENERTLDFHDSNVNNLYDKVRLQLKDNARELGNGCFEFYHKCDNECMESVRNGTYDYPQYSEEARLNREEISGVKLESMGVYQILSIYSTVASSLALAIMIAGLSFWMCSNGSLQCRICI

SEQ ID NO: 6 - protein, 566 aa, Influenza virus A
  influenza virus A hemagglutinin subtype H6
MIAIIVVAILATAGRSDKICIGYHANNSTTQIDTILEKNVTVTHSVELLENQKEERFCKILKKAPLDLKGCTIEGWILGNPQCDLLLGDQSWSYIVERPTAQNGICYPGVLNEVEELKALIGSGERVERFEMFPKSTWTGVDTSSGVTRACPYNSGSSFYRNLLWIIKTKSAAYSVIKGAYNNTGNQPILYFWGVHHPPDTNEQNTLYGSGDRYVRMGTESMNFAKSPEIAARPAVNGQRGRIDYYWSILKPGETLNVESNGNLIAPWYAFRFVSTSNKGAVFKSNLPIENCDATCQTVAGVLRTNKTFQNVSPLWIGECPKYVKSESLRLATGLRNVPQIETRGLFGAIAGFIEGGWTGMIDGWYGYHHENSQGSGYAADRESTQKAVDGITNKVNSIIDKMNTQFEAVDHEFSNLERRIDNLNKRMEDGFLDVWTYNAELLVLLENERTLDLHDANVKNLYERVKSQLRDNAMILGNGCFEFWHKCDDECMESVKNGTYDYPKYQDESKLNRQEIESVKLESLGVYQILAIYSTVSSSLVLVGLIIAVGLWMCSNGSMQCRICI

SEQ ID NO: 7 - protein, 563 aa, Influenza virus A
  influenza virus A hemagglutinin subtype H7
MNTQILVFALVAVIPTNADKICLGHHAVSNGTKVNTLTERGVEVVNATETVERTNIPKICSKGKRTTDLGQCGLLGTITGPPQCDQFLEFSADLIIERREGNDVCYPGKFVNEEALRQILRGSGGIDKETMGFTYSGIRTNGTTSACRRSGSSFYAEMEWLLSNTDNASFPQMTKSYKNTRRESALIVWGIHHSGSTTEQTKLYGSGNKLITVGSSKYHQSFVPSPGTRPQINGQSGRIDFHWLILDPNDTVTFSFNGAFIAPNRASFLRGKSMGIQSDVQVDANCEGECYHSGGTITSRLPFQNINSRAVGKCPRYVKQESLLLATGMKNVPEPSKKRKKRGLFGAIAGFIENGWEGLVDGWYGFRHQNAQGEGTAADYKSTQSAIDQITGKLNRLIEKTNQQFELIDNEFTEVEKQIGNLINWTKDSITEVWSYNAELIVAMENQHTIDLADSEMNRLYERVRKQLRENAEEDGTGCFEIFHKCDDDCMASIRNNTYDHSKYREEAMQNRIQIDPVKLSSGYKDVILWFSFGASCFLLLAIAMGLVFICVKNGNMRCTICI

SEQ ID NO: 8 - protein, 565 aa, Influenza virus A
  influenza virus A hemagglutinin subtype H8
MEKFIAIATLASTNAYDRICIGYQSNNSTDTVNTLIEQNVPVTQTMELVETEKHPAYCNTDLGAPLELRDCKIEAVIYGNPKCDIHLKDQGWSYIVERPSAPEGMCYPGSVENLEELRFVFSSAASYKRIRLFDYSRWNVTRSGTSKACNASTGGQSFYRSINWLTKKEPDTYDFNEGAYVNNEDGDIIFLWGIHHPPDTKEQTTLYKNANTLSSVTTNTINRSFQPNIGPRPLVRGQQGRMDYYWGILKRGETLKIRTNGNLIAPEFGYLLKGESYGRIIQNEDIPIGNCNTKCQTYAGAINSSKPFQNASRHYMGECPKYVKKASLRLAVGLRNTPSVEPRGLFGAIAGFIEGGWSGMIDGWYGFHHSNSEGTGMAADQKSTQEAIDKITNKVNNIVDKMNREFEVVNHEFSEVEKRINMINDKIDDQIEDLWAYNAELLVLLENQKTLDEHDSNVKNLFDEVKRRLSANAIDAGNGCFDILHKCDNECMETIKNGTYDHKEYEEEAKLERSKINGVKLEENTTYKILSIYSTVAASLCLAILIAGGLILGMQNGSCRCMFCI

SEQ ID NO: 9 - protein, 560 aa, Influenza virus A
  influenza virus A hemagglutinin subtype H9
METKAIIAALLMVTAANADKICIGYQSTNSTETVDTLTESNVPVTHTKELLHTEHNGMLCATDLGHPLILDTCTIEGLIYGNPSCDILLGGKEWSYIVERSSAVNGMCYPGNVENLEELRSLFSSAKSYKRIQIFPDKTWNVTYSGTSRACSNSFYRSMRWLTHKSNSYPFQNAHYTNNERENILFMWGIHHPPTDTEQTDLYKNADTTTSVTTEDINRTFKPVIGPRPLVNGQQGRIDYYWSVLKPGQTLRIRSNGNLIAPWYGHVLTGESHGRILKTDLNNGNCVVQCQTEKGGLNTTLPFHNISKYAFGNCPKYVGVKSLKLPVGLRNVPAVSSRGLFGAIAGFIEGGWPGLVAGWYGFQHSNDQGVGMAADKGSTQKAIDKITSKVNNIIDKMNKQYEVIDHEFNELEARLNMINNKIDDQIQDIWAYNAELLVLLENQKTLDEHDANVNNLYNKVKRALGSNAVEDGNGCFELYHKCDDQCMETIRNGTYDRQKYQEESRLERQKIEGVKLESEGTYKILTIYSTVASSLVLAMGFAAFLFWAMSNGSCRCNICI

SEQ ID NO: 10 - protein, 561 aa, Influenza virus A
  influenza virus A hemagglutinin subtype H10
MYKVVVIIALLGAVKGLDRICLGHHAVANGTIVKTLTNEQEEVTNATETVESTNLNKLCMKGRSYKDLGNCHPVGMLIGTPVCDPHLTGTWDTLIERENAIAHCYPGATINEEALRQKIMESGGISKMSTGFTYGSSITSAGTTKACMRNGGDSFYAELKWLVSKTKGQNFPQTTNTYRNTDTAEHLIIWGIHHPSSTQEKNDLYGTQSLSISVESSTYQNNFVPVVGARPQVNGQSGRIDFHWTLVQPGDNITFSDNGGLIAPSRVSKLTGRDLGIQSEALIDNSCESKCFWRGGSINTKLPFQNLSPRTVGQCPKYVNQRSLLLATGMRNVPEVVQGRGLFGAIAGFIENGWEGMVDGWYGFRHQNAQGTGQAADYKSTQAAIDQITGKLNRLIEKTNTEFESIESEFSETEHQIGNVINWTKDSITDIWTYNAELLVAMENQHTIDMADSEMLNLYERVRKQLRQNAEEDGKGCFEIYHTCDDSCMESIRNNTYDHSQYREEALLNRLNINPVKLSSGYKDIILWFSFGESCFVLLAVVMGLVFFCLKNGNMRCTICI

SEQ ID NO: 11 - protein, 565 aa, Influenza virus A
  influenza virus A hemagglutinin subtype H11
MEKTLLFAAIFLCVKADEICIGYLSNNSTDKVDTIIENNVTVTSSVELVETEHTGSFCSINGKQPISLGDCSFAGWILGNPMCDELIGKTSWSYIVEKPNPTNGICYPGTLESEEELRLKFSGVLEFNKFEVFTSNGWGAVNSGVGVTAACKFGGSNSFFRNMVWLIHQSGTYPVIKRTFNNTKGRDVLIVWGIHHPATLTEHQDLYKKDSSYVAVGSETYNRRFTPEINTRPRVNGQAGRMTFYWKIVKPGESITFESNGAFLAPRYAFEIVSVGNGKLFRSELNIESCSTKCQTEIGGINTNKSFHNVHRNTIGDCPKYVNVKSLKLATGPRNVPAIASRGLFGAIAGFIEGGWPGLINGWYGFQHRDEEGTGIAADKESTQKAIDQITSKVNNIVDRMNTNFESVQHEFSEIEERINQLSKHVDDSVVDIWSYNAQLLVLLENEKTLDLHDSNVRNLHEKVRRMLKDNAKDEGNGCFTFYHKCDNKCIERVRNGTYDHKEFEEESKINRQEIEGVKLDSSGNVYKILSIYSCIASSLVLAALIMGFMFWACSNGSCRCTICI

SEQ ID NO: 12 - protein, 564 aa, Influenza virus A
  influenza virus A hemagglutinin subtype H12
MEKFIILSTVLAASFAYDKICIGYQTNNSTETVNTLSEQNVPVTQVEELVHRGIDPILCGTELGSPLVLDDCSLEGLILGNPKCDLYLNGREWSYIVERPKEMEGVCYPGSIENQEELRSLFSSIKKYERVKMFDFTKWNVTYTGTSKACNNTSNQGSFYRSMRWLTLKSGQFPVQTDEYKNTRDSDIVFTWAIHHPPTSDEQVKLYKNPDTLSSVTTVEINRSFKPNIGPRPLVRGQQGRMDYYWAVLKPGQTVKIQTNGNLIAPEYGHLITGKSHGRILKNNLPMGQCVTECQLNEGVMNTSKPFQNTSKHYIGKCPKYIPSGSLKLAIGLRNVPQVQDRGLFGAIAGFIEGGWPGLVAGWYGFQHQNAEGTGIAADRDSTQRAIDNMQNKLNNVIDKMNKQFEVVNHEFSEVESRINMINSKIDDQITDIWAYNAELLVLLENQKTLDEHDANVRNLHDRVRRVLRENAIDTGDGCFEILHKCDNNCMDTIRNGTYNHKEYEEESKIERQKVNGVKLEENSTYKILSIYSSVASSLVLLLMIIGGFIFGCQNGNVRCTFCI

SEQ ID NO: 13 - protein, 566 aa, Influenza virus A
  influenza virus A hemagglutinin subtype H13
MALNVIATLTLISVCVHADRICVGYLSTNSSERVDTLLENGVPVTSSIDLIETNHTGTYCSLNGVSPVHLGDCSFEGWIVGNPACTSNFGIREWSYLIEDPAAPHGLCYPGELNNNGELRHLFSGIRSFSRTELIPPTSWGEVLDGTTSACRDNTGTNSFYRNLVWFIKKNTRYPVISKTYNNTTGRDVLVLWGIHHPVSVDETKTLYVNSDPYTLVSTKSWSEKYKLETGVRPGYNGQRSWMKIYWSLIHPGEMITFESNGGFLAPRYGYIIEEYGKGRIFQSRIRMSRCNTKCQTSVGGINTNRTFQNIDKNALGDCPKYIKSGQLKLATGLRNVPAISNRGLFGAIAGFIEGGWPGLINGWYGFQHQNEQGTGIAADKESTQKAIDQITTKINNIIDKMNGNYDSIRGEFNQVEKRINMLADRIDDAVTDIWSYNAKLLVLLENDKTLDMHDANVKNLHEQVRRELKDNAIDEGNGCFELLHKCNDSCMETIRNGTYDHTEYAEESKLKRQEIDGIKLKSEDNVYKALSIYSCIASSVVLVGLILSFIMWACSSGNCRFNVCI

SEQ ID NO: 14 - protein, 568 aa, Influenza virus A
  influenza virus A hemagglutinin subtype H14
MIALILVALALSHTAYSQITNGTTGNPIICLGHHAVENGTSVKTLTDNHVEVVSAKELVETNHTDELCPSPLKLVDGQDCHLINGALGSPGCDRLQDTTWDVFIERPTAVDTCYPFDVPDYQSLRSILASSGSLEFIAEQFTWNGVKVDGSSSACLRGGRNSFFSRLNWLTKATNGNYGPINVTKENTGSYVRLYLWGVHHPSSDNEQTDLYKVATGRVTVSTRSDQISIVPNIGSRPRVRNQSGRISIYWTLVNPGDSIIFNSIGNLIAPRGHYKISKSTKSTVLKSDKRIGSCTSPCLTDKGSIQSDKPFQNVSRIAIGNCPKYVKQGSLMLATGMRNIPGKQAKGLFGAIAGFIENGWQGLIDGWYGFRHQNAEGTGTAADLKSTQAAIDQINGKLNRLIEKTNEKYHQIEKEFEQVEGRIQDLEKYVEDTKIDLWSYNAELLVALENQHTIDVTDSEMNKLFERVRRQLRENAEDQGNGCFEIFHQCDNNCIESIRNGTYDHNIYRDEAINNRIKINPVTLTMGYKDIILWISFSMSCFVFVALILGFVLWACQNGNIRCQICI

SEQ ID NO: 15 - protein, 570 aa, Influenza virus A
  influenza virus A hemagglutinin subtype H15
MNTQIIVILVLGLSMVKSDKICLGHHAVANGTKVNTLTERGVEVVNATETVEITGIDKVCTKGKKAVDLGSCGILGTIIGPPQCDLHLEFKADLIIERRNSSDICYPGRFTNEEALRQIIRESGGIDKESMGFRYSGIRTDGATSACKRTVSSFYSEMKWLSSSMNNQVFPQLNQTYRNTRKEPALIVWGVHHSSSLDEQNKLYGTGNKLITVGSSKYQQSFSPSPGARPKVNGQAGRIDFHWMLLDPGDTVTFTFNGAFIAPDRATFLRSNAPSGIEYNGKSLGIQSDAQIDESCEGECFYSGGTINSPLPFQNIDSRAVGKCPRYVKQSSLPLALGMKNVPEKIRTRGLFGAIAGFIENGWEGLIDGWYGFRHQNAQGQGTAADYKSTQAAIDQITGKLNRLIEKTNKQFELIDNEFTEVEQQIGNVINWTRDSLTEIWSYNAELLVAMENQHTIDLADSEMNKLYERVRRQLRENAEEDGTGCFEIFHRCDDQCMESIRNNTYNHTEYRQEALQNRIMINPVKLSSGYKDVILWFSFGASCVMLLAIAMGLIFMCVKNGNLRCTICI

SEQ ID NO: 16 - protein, 565 aa, Influenza virus A
  influenza virus A hemagglutinin subtype H16
MMIKVLYFLIIVLGRYSKADKICIGYLSNNSSDTVDTLTENGVPVTSSVDLVETNHTGTYCSLNGISPIHLGDCSFEGWIVGNPSCATNINIREWSYLIEDPNAPNKFCYPGELDNNGELRHLFSGVNSFSRTELINPSKWGNVLDGVTASCLDRGASSFYRNLVWIVKKDEKYPVIKGDYNNTTGRDVLVLWGIHHPDTETTATNLYVNKNPYTLVSTKEWSKRYELEIGTRIGDGQRSWMKLYWHLMHPGERIMFESNGGLIAPRYGYIIEKYGTGRIFQSGVRMARCNTKCQTSLGGINTNKTFQNIERNALGDCPKYIKSGQLKLATGLRNVPSIGERGLFGAIAGFIEGGWPGLINGWYGFQHQNEQGTGIAADKASTQKAINEITTKINNIIEKMNGNYDSIRGEFNQVEKRINMLADRVDDAVTDIWSYNAKLLVLLENDRTLDLHDANVRNLHDQVKRALKSNAIDEGDGCFNLLHKCNDSCMETIRNGTYNHEDYREESQLKRQEIEGIKLKTEDNVYKVLSIYSCIASSIVLVGLILAFIMWACSNGSCRFNVCI

SEQ ID NO: 17 - protein, 342 aa, Influenza virus B
  influenza B virus hemagglutinin (in Fig. 3)
DRICTGITSSNSPHVVKTATQGEVNVTGVIPLTTTPTKSHFANLKGTQTRGKLCPNCLNCTDLDVALGRPKCMGTIPSAKASILHEVKPVTSGCFPIMHDRTKIRQLPNLLRGYENIRLSARNVTNAETAPGGPYIVGTSGSCPNVTNGNGFFATMAWAVPKNKTATNPLTVEVPYICTKGEDQITVWGFHSDDETQMVKLYGDSKPQKFTSSANGVTTHYVSQIGGFPNQAEDEGLPQSGRIVVDYMVQKPGKTGTIAYQRGVLLPQKVWCASGRSKVIKGSLPLIGEADCLHEKYGGLNKSKPYYTGEHAKAIGNCPIWVKTPLKLANGTKYRPPAKLLK

SEQ ID NO: 18 - protein, 17 aa, Influenza virus A
  influenza A HA subtype H1 signal peptides
MKANLLVLLCALAAADA

SEQ ID NO: 19 - protein, 15 aa, Influenza virus A
  influenza A HA subtype H2 signal peptides
MAIIYLILLFTAVRG

SEQ ID NO: 20 - protein, 16 aa, Influenza virus A
  influenza A HA subtype H3 signal peptides
MKTIIALSYIFCLALG

SEQ ID NO: 21 - protein, 16 aa, Influenza virus A
  influenza A HA subtype H4 signal peptides
MLSIVILFLLIAENSS

SEQ ID NO: 22 - protein, 16 aa, Influenza virus A
  influenza A HA subtype H5 signal peptides
MERIVLLLAIVSLVKS

SEQ ID NO: 23 - protein, 16 aa, Influenza virus A
  influenza A HA subtype H6 signal peptides
MIAIIVVAILATAGRS

SEQ ID NO: 24 - protein, 18 aa, Influenza virus A
  influenza A HA subtype H7 signal peptides
MNTQILVFALVAVIPTNA

SEQ ID NO: 25 - protein, 16 aa, Influenza virus A
  influenza A HA subtype H8 signal peptides
MEKFIAIATLASTNAY

SEQ ID NO: 26 - protein, 18 aa, Influenza virus A
  influenza A HA subtype H9 signal peptides
METKAIIAALLMVTAANA

SEQ ID NO: 27 - protein, 16 aa, Influenza virus A
  influenza A HA subtype H10 signal peptides
MYKVVVIIALLGAVKG

SEQ ID NO: 28 - protein, 16 aa, Influenza virus A
  influenza A HA subtype H11 signal peptides
MEKTLLFAAIFLCVKA

SEQ ID NO: 29 - protein, 17 aa, Influenza virus A
  influenza A HA subtype H12 signal peptides
MEKFIILSTVLAASFAY

SEQ ID NO: 30 - protein, 18 aa, Influenza virus A
  influenza A HA subtype H13 signal peptides
MALNVIATLTLISVCVHA

SEQ ID NO: 31 - protein, 17 aa, Influenza virus A
  influenza A HA subtype H14 signal peptides
MIALILVALALSHTAYS

SEQ ID NO: 32 - protein, 18 aa, Influenza virus A
  influenza A HA subtype H15 signal peptides
MNTQIIVILVLGLSMVKS

SEQ ID NO: 33 - protein, 19 aa, Influenza virus A
  influenza A HA subtype H16 signal peptides
MMIKVLYFLIIVLGRYSKA

SEQ ID NO: 34 - protein, 42 aa, Influenza virus A
  influenza A HA subtype H1 N-terminal stem segment
DTICIGYHANNSTDTVDTVLEKNVTVTHSVNLLEDSHNGKLC

SEQ ID NO: 35 - protein, 42 aa, Influenza virus A
  influenza A HA subtype H2 N-terminal stem segment
DQICIGYHSNNSTEKVDTILERNVTVTHAQNILEKTHNGKLC

SEQ ID NO: 36 - protein, 52 aa, Influenza virus A
  influenza A HA subtype H3 N-terminal stem segment
QDLPGNDNSTATLCLGHHAVPNGTLVKTITDDQIEVTNATELVQSSSTGKIC

SEQ ID NO: 37 - protein, 48 aa, Influenza virus A
  influenza A HA subtype H4 N-terminal stem segment
QNYTGNPVICMGHHAVANGTMVKTLADDQVEVVTAQELVESQNLPELC

SEQ ID NO: 38 - protein, 42 aa, Influenza virus A
  influenza A HA subtype H5 N-terminal stem segment
DQICIGYHANKSTKQVDTIMEKNVTVTHAQDILERTHNGKLC

SEQ ID NO: 39 - protein, 42 aa, Influenza virus A
  influenza A HA subtype H6 N-terminal stem segment
DKICIGYHANNSTTQIDTILEKNVTVTHSVELLENQKEERFC

SEQ ID NO: 40 - protein, 42 aa, Influenza virus A
  influenza A HA subtype H7 N-terminal stem segment
DKICLGHHAVSNGTKVNTLTERGVEVVNATETVERTNIPKIC

SEQ ID NO: 41 - protein, 42 aa, Influenza virus A
  influenza A HA subtype H8 N-terminal stem segment
DRICIGYQSNNSTDTVNTLIEQNVPVTQTMELVETEKHPAYC

SEQ ID NO: 42 - protein, 42 aa, Influenza virus A
  influenza A HA subtype H9 N-terminal stem segment
DKICIGYQSTNSTETVDTLTESNVPVTHTKELLHTEHNGMLC

SEQ ID NO: 43 - protein, 43 aa, Influenza virus A
  influenza A HA subtype H10 N-terminal stem segment
LDRICLGHHAVANGTIVKTLTNEQEEVTNATETVESTNLNKLC

SEQ ID NO: 44 - protein, 42 aa, Influenza virus A
  influenza A HA subtype H11 N-terminal stem segment
DEICIGYLSNNSTDKVDTIIENNVTVTSSVELVETEHTGSFC

SEQ ID NO: 45 - protein, 42 aa, Influenza virus A
  influenza A HA subtype H12 N-terminal stem segment
DKICIGYQTNNSTETVNTLSEQNVPVTQVEELVHRGIDPILC

SEQ ID NO: 46 - protein, 42 aa, Influenza virus A
  influenza A HA subtype H13 N-terminal stem segment
DRICVGYLSTNSSERVDTLLENGVPVTSSIDLIETNHTGTYC

SEQ ID NO: 47 - protein, 51 aa, Influenza virus A
  influenza A HA subtype H14 N-terminal stem segment
QITNGTTGNPIICLGHHAVENGTSVKTLTDNHVEVVSAKELVETNHTDELC

SEQ ID NO: 48 - protein, 42 aa, Influenza virus A
  influenza A HA subtype H15 N-terminal stem segment
DKICLGHHAVANGTKVNTLTERGVEVVNATETVEITGIDKVC

SEQ ID NO: 49 - protein, 42 aa, Influenza virus A
  influenza A HA subtype H16 N-terminal stem segment
DKICIGYLSNNSSDTVDTLTENGVPVTSSVDLVETNHTGTYC

SEQ ID NO: 50 - protein, 53 aa, Influenza virus A
  influenza A HA subtype H1 C-terminal stem segment
CNTKCQTPLGAINSSLPYQNIHPVTIGECPKYVRSAKLRMVTGLRNNPSIQSR

SEQ ID NO: 51 - protein, 53 aa, Influenza virus A
  influenza A HA subtype H2 C-terminal stem segment
CETKCQTPLGAINTTLPFHNVHPLTIGECPKYVKSERLVLATGLRNVPQIESR

SEQ ID NO: 52 - protein, 53 aa, Influenza virus A
  influenza A HA subtype H3 C-terminal stem segment
CISECITPNGSIPNDKPFQNVNKITYGACPKYVKQNTLKLATGMRNVPEKQTR

SEQ ID NO: 53 - protein, 53 aa, Influenza virus A
  influenza A HA subtype H4 C-terminal stem segment
CVSKCHTDKGSLSTTKPFQNISRIAVGDCPRYVKQGSLKLATGMRNIPEKASR

SEQ ID NO: 54 - protein, 53 aa, Influenza virus A
  influenza A HA subtype H5 C-terminal stem segment
CDTKCQTPVGEINSSMPFHNIHPHTIGECPKYVKSDRLVLATGLRNVPQRKKR

SEQ ID NO: 55 - protein, 53 aa, Influenza virus A
  influenza A HA subtype H6 C-terminal stem segment
CDATCQTVAGVLRTNKTFQNVSPLWIGECPKYVKSESLRLATGLRNVPQIETR

SEQ ID NO: 56 - protein, 57 aa, Influenza virus A
  influenza A HA subtype H7 C-terminal stem segment
CEGECYHSGGTITSRLPFQNINSRAVGKCPRYVKQESLLLATGMKNVPEPSKKRKKR

SEQ ID NO: 57 - protein, 53 aa, Influenza virus A
  influenza A HA subtype H8 C-terminal stem segment
CNTKCQTYAGAINSSKPFQNASRHYMGECPKYVKKASLRLAVGLRNTPSVEPR

SEQ ID NO: 58 - protein, 53 aa, Influenza virus A
  influenza A HA subtype H9 C-terminal stem segment
CVVQCQTEKGGLNTTLPFHNISKYAFGNCPKYVGVKSLKLPVGLRNVPAVSSR

SEQ ID NO: 59 - protein, 54 aa, Influenza virus A
  influenza A HA subtype H10 C-terminal stem segment
CESKCFWRGGSINTKLPFQNLSPRTVGQCPKYVNQRSLLLATGMRNVPEVVQGR

SEQ ID NO: 60 - protein, 53 aa, Influenza virus A
  influenza A HA subtype H11 C-terminal stem segment
CSTKCQTEIGGINTNKSFHNVHRNTIGDCPKYVNVKSLKLATGPRNVPAIASR

SEQ ID NO: 61 - protein, 53 aa, Influenza virus A
  influenza A HA subtype H12 C-terminal stem segment
CVTECQLNEGVMNTSKPFQNTSKHYIGKCPKYIPSGSLKLAIGLRNVPQVQDR

SEQ ID NO: 62 - protein, 53 aa, Influenza virus A
  influenza A HA subtype H13 C-terminal stem segment
CNTKCQTSVGGINTNRTFQNIDKNALGDCPKYIKSGQLKLATGLRNVPAISNR

SEQ ID NO: 63 - protein, 53 aa, Influenza virus A
  influenza A HA subtype H14 C-terminal stem segment
CTSPCLTDKGSIQSDKPFQNVSRIAIGNCPKYVKQGSLMLATGMRNIPGKQAK

SEQ ID NO: 64 - protein, 54 aa, Influenza virus A
  influenza A HA subtype H15 C-terminal stem segment
CEGECFYSGGTINSPLPFQNIDSRAVGKCPRYVKQSSLPLALGMKNVPEKIRTR

SEQ ID NO: 65 - protein, 53 aa, Influenza virus A
  influenza A HA subtype H16 C-terminal stem segment
CNTKCQTSLGGINTNKTFQNIERNALGDCPKYIKSGQLKLATGLRNVPSIGER

SEQ ID NO: 66 - protein, 222 aa, Influenza virus A
  influenza A HA subtype H1 HA2 domain
GLFGAIAGFIEGGWTGMIDGWYGYHHQNEQGSGYAADQKSTQNAINGITNKVNTVIEKMNIQFTAVGKEFNKLEKRMENLNKKVDDGFLDIWTYNAELLVLLENERTLDFHDSNVKNLYEKVKSQLKNNAKEIGNGCFEFYHKCDNECMESVRNGTYDYPKYSEESKLNREKVDGVKLESMGIYQILAIYSTVASSLVLLVSLGAISFWMCSNGSLQCRICI

SEQ ID NO: 67 - protein, 222 aa, Influenza virus A
  influenza A HA subtype H2 HA2 domain
GLFGAIAGFIEGGWQGMIDGWYGYHHSNDQGSGYAADKESTQKAIDGITNRVNSVIEKMNTQFEAVGKEFSNLEKRLENLNKKMEDGFLDVWTYNAELLVLMENERTLDFHDSNVKNLYDRVRMQLRDNAKELGNGCFEFYHKCDDECMNSVKNGTYDYPKYEEESKLNRNEIKGVKLSNMGVYQILAIYATVAGSLSLAIMIAGISLWMCSNGSLQCRICI

SEQ ID NO: 68 - protein, 221 aa, Influenza virus A
  influenza A HA subtype H3 HA2 domain
GLFGAIAGFIENGWEGMIDGWYGFRHQNSEGTGQAADLKSTQAAIDQINGKLNRVIEKTNEKFHQIEKEFSEVEGRIQDLEKYVEDTKIDLWSYNAELLVALENQHTIDLTDSEMNKLFEKTRRQLRENAEDMGNGCFKIYHKCDNACIESIRNGTYDHDVYRDEALNNRFQIKGVELKSGYKDWILWISFAISCFLLCVVLLGFIMWACQRGNIRCNICI

SEQ ID NO: 69 - protein, 221 aa, Influenza virus A
  influenza A HA subtype H4 HA2 domain
GLFGAIAGFIENGWQGLIDGWYGFRHQNAEGTGTAADLKSTQAAIDQINGKLNRLIEKTNDKYHQIEKEFEQVEGRIQDLENYVEDTKIDLWSYNAELLVALENQHTIDVTDSEMNKLFERVRRQLRENAEDKGNGCFEIFHKCDNNCIESIRNGTYDHDIYRDEAINNRFQIQGVKLTQGYKDIILWISFSISCFLLVALLLAFILWACQNGNIRCQICI

SEQ ID NO: 70 - protein, 222 aa, Influenza virus A
  influenza A HA subtype H5 HA2 domain
GLFGAIAGFIEGGWQGMVDGWYGYHHSNEQGSGYAADKESTQKAIDGITNKVNSIIDKMNTRFEAVGKEFNNLERRVENLNKKMEDGFLDVWTYNVELLVLMENERTLDFHDSNVNNLYDKVRLQLKDNARELGNGCFEFYHKCDNECMESVRNGTYDYPQYSEEARLNREEISGVKLESMGVYQILSIYSTVASSLALAIMIAGLSFWMCSNGSLQCRICI

SEQ ID NO: 71 - protein, 222 aa, Influenza virus A
  influenza A HA subtype H6 HA2 domain
GLFGAIAGFIEGGWTGMIDGWYGYHHENSQGSGYAADRESTQKAVDGITNKVNSIIDKMNTQFEAVDHEFSNLERRIDNLNKRMEDGFLDVWTYNAELLVLLENERTLDLHDANVKNLYERVKSQLRDNAMILGNGCFEFWHKCDDECMESVKNGTYDYPKYQDESKLNRQEIESVKLESLGVYQILAIYSTVSSSLVLVGLIIAVGLWMCSNGSMQCRICI

SEQ ID NO: 72 - protein, 221 aa, Influenza virus A
  influenza A HA subtype H7 HA2 domain
GLFGAIAGFIENGWEGLVDGWYGFRHQNAQGEGTAADYKSTQSAIDQITGKLNRLIEKTNQQFELIDNEFTEVEKQIGNLINWTKDSITEVWSYNAELIVAMENQHTIDLADSEMNRLYERVRKQLRENAEEDGTGCFEIFHKCDDDCMASIRNNTYDHSKYREEAMQNRIQIDPVKLSSGYKDVILWFSFGASCFLLLAIAMGLVFICVKNGNMRCTICI

SEQ ID NO: 73 - protein, 222 aa, Influenza virus A
  influenza A HA subtype H8 HA2 domain
GLFGAIAGFIEGGWSGMIDGWYGFHHSNSEGTGMAADQKSTQEAIDKITNKVNNIVDKMNREFEVVNHEFSEVEKRINMINDKIDDQIEDLWAYNAELLVLLENQKTLDEHDSNVKNLFDEVKRRLSANAIDAGNGCFDILHKCDNECMETIKNGTYDHKEYEEEAKLERSKINGVKLEENTTYKILSIYSTVAASLCLAILIAGGLILGMQNGSCRCMFCI

SEQ ID NO: 74 - protein, 222 aa, Influenza virus A
  influenza A HA subtype H9 HA2 domain
GLFGAIAGFIEGGWPGLVAGWYGFQHSNDQGVGMAADKGSTQKAIDKITSKVNNIIDKMNKQYEVIDHEFNELEARLNMINNKIDDQIQDIWAYNAELLVLLENQKTLDEHDANVNNLYNKVKRALGSNAVEDGNGCFELYHKCDDQCMETIRNGTYDRQKYQEESRLERQKIEGVKLESEGTYKILTIYSTVASSLVLAMGFAAFLFWAMSNGSCRCNICI

SEQ ID NO: 75 - protein, 221 aa, Influenza virus A
  influenza A HA subtype H10 HA2 domain
GLFGAIAGFIENGWEGMVDGWYGFRHQNAQGTGQAADYKSTQAAIDQITGKLNRLIEKTNTEFESIESEFSETEHQIGNVINWTKDSITDIWTYNAELLVAMENQHTIDMADSEMLNLYERVRKQLRQNAEEDGKGCFEIYHTCDDSCMESIRNNTYDHSQYREEALLNRLNINPVKLSSGYKDIILWFSFGESCFVLLAVVMGLVFFCLKNGNMRCTICI

SEQ ID NO: 76 - protein, 223 aa, Influenza virus A
  influenza A HA subtype H11 HA2 domain
GLFGAIAGFIEGGWPGLINGWYGFQHRDEEGTGIAADKESTQKAIDQITSKVNNIVDRMNTNFESVQHEFSEIEERINQLSKHVDDSVVDIWSYNAQLLVLLENEKTLDLHDSNVRNLHEKVRRMLKDNAKDEGNGCFTFYHKCDNKCIERVRNGTYDHKEFEEESKINRQEIEGVKLDSSGNVYKILSIYSCIASSLVLAALIMGFMFWACSNGSCRCTICI

SEQ ID NO: 77 - protein, 222 aa, Influenza virus A
  influenza A HA subtype H12 HA2 domain
GLFGAIAGFIEGGWPGLVAGWYGFQHQNAEGTGIAADRDSTQRAIDNMQNKLNNVIDKMNKQFEVVNHEFSEVESRINMINSKIDDQITDIWAYNAELLVLLENQKTLDEHDANVRNLHDRVRRVLRENAIDTGDGCFEILHKCDNNCMDTIRNGTYNHKEYEEESKIERQKVNGVKLEENSTYKILSIYSSVASSLVLLLMIIGGFIFGCQNGNVRCTFCI

SEQ ID NO: 78 - protein, 223 aa, Influenza virus A
  influenza A HA subtype H13 HA2 domain
GLFGAIAGFIEGGWPGLINGWYGFQHQNEQGTGIAADKESTQKAIDQITTKINNIIDKMNGNYDSIRGEFNQVEKRINMLADRIDDAVTDIWSYNAKLLVLLENDKTLDMHDANVKNLHEQVRRELKDNAIDEGNGCFELLHKCNDSCMETIRNGTYDHTEYAEESKLKRQEIDGIKLKSEDNVYKALSIYSCIASSVVLVGLILSFIMWACSSGNCRFNVCI

SEQ ID NO: 79 - protein, 221 aa, Influenza virus A
  influenza A HA subtype H14 HA2 domain
GLFGAIAGFIENGWQGLIDGWYGFRHQNAEGTGTAADLKSTQAAIDQINGKLNRLIEKTNEKYHQIEKEFEQVEGRIQDLEKYVEDTKIDLWSYNAELLVALENQHTIDVTDSEMNKLFERVRRQLRENAEDQGNGCFEIFHQCDNNCIESIRNGTYDHNIYRDEAINNRIKINPVTLTMGYKDIILWISFSMSCFVFVALILGFVLWACQNGNIRCQICI

SEQ ID NO: 80 - protein, 221 aa, Influenza virus A
  influenza A HA subtype H15 HA2 domain
GLFGAIAGFIENGWEGLIDGWYGFRHQNAQGQGTAADYKSTQAAIDQITGKLNRLIEKTNKQFELIDNEFTEVEQQIGNVINWTRDSLTEIWSYNAELLVAMENQHTIDLADSEMNKLYERVRRQLRENAEEDGTGCFEIFHRCDDQCMESIRNNTYNHTEYRQEALQNRIMINPVKLSSGYKDVILWFSFGASCVMLLAIAMGLIFMCVKNGNLRCTICI

SEQ ID NO: 81 - protein, 223 aa, Influenza virus A
  influenza A HA subtype H16 HA2 domain
GLFGAIAGFIEGGWPGLINGWYGFQHQNEQGTGIAADKASTQKAINEITTKINNIIEKMNGNYDSIRGEFNQVEKRINMLADRVDDAVTDIWSYNAKLLVLLENDRTLDLHDANVRNLHDQVKRALKSNAIDEGDGCFNLLHKCNDSCMETIRNGTYNHEDYREESQLKRQEIEGIKLKTEDNVYKVLSIYSCIASSIVLVGLILAFIMWACSNGSCRFNVCI

SEQ ID NO: 82 - protein, 180 aa, Influenza virus A
  influenza A HA2 domain subtype H1 stem domain
GLFGAIAGFIEGGWTGMIDGWYGYHHQNEQGSGYAADQKSTQNAINGITNKVNTVIEKMNIQFTAVGKEFNKLEKRMENLNKKVDDGFLDIWTYNAELLVLLENERTLDFHDSNVKNLYEKVKSQLKNNAKEIGNGCFEFYHKCDNECMESVRNGTYDYPKYSEESKLNREKVDGVKLES

SEQ ID NO: 83 - protein, 180 aa, Influenza virus A
  influenza A HA2 domain subtype H2 stem domain
GLFGAIAGFIEGGWQGMIDGWYGYHHSNDQGSGYAADKESTQKAIDGITNRVNSVIEKMNTQFEAVGKEFSNLEKRLENLNKKMEDGFLDVWTYNAELLVLMENERTLDFHDSNVKNLYDRVRMQLRDNAKELGNGCFEFYHKCDDECMNSVKNGTYDYPKYEEESKLNRNEIKGVKLSN

SEQ ID NO: 84 - protein, 179 aa, Influenza virus A
  influenza A HA2 domain subtype H3 stem domain
GLFGAIAGFIENGWEGMIDGWYGFRHQNSEGTGQAADLKSTQAAIDQINGKLNRVIEKTNEKFHQIEKEFSEVEGRIQDLEKYVEDTKIDLWSYNAELLVALENQHTIDLTDSEMNKLFEKTRRQLRENAEDMGNGCFKIYHKCDNACIESIRNGTYDHDVYRDEALNNRFQIKGVELK

SEQ ID NO: 85 - protein, 179 aa, Influenza virus A
  influenza A HA2 domain subtype H4 stem domain
GLFGAIAGFIENGWQGLIDGWYGFRHQNAEGTGTAADLKSTQAAIDQINGKLNRLIEKTNDKYHQIEKEFEQVEGRIQDLENYVEDTKIDLWSYNAELLVALENQHTIDVTDSEMNKLFERVRRQLRENAEDKGNGCFEIFHKCDNNCIESIRNGTYDHDIYRDEAINNRFQIQGVKLT

SEQ ID NO: 86 - protein, 180 aa, Influenza virus A
  influenza A HA2 domain subtype H5 stem domain
GLFGAIAGFIEGGWQGMVDGWYGYHHSNEQGSGYAADKESTQKAIDGITNKVNSIIDKMNTRFEAVGKEFNNLERRVENLNKKMEDGFLDVWTYNVELLVLMENERTLDFHDSNVNNLYDKVRLQLKDNARELGNGCFEFYHKCDNECMESVRNGTYDYPQYSEEARLNREEISGVKLES

SEQ ID NO: 87 - protein, 180 aa, Influenza virus A
  influenza A HA2 domain subtype H6 stem domain
GLFGAIAGFIEGGWTGMIDGWYGYHHENSQGSGYAADRESTQKAVDGITNKVNSIIDKMNTQFEAVDHEFSNLERRIDNLNKRMEDGFLDVWTYNAELLVLLENERTLDLHDANVKNLYERVKSQLRDNAMILGNGCFEFWHKCDDECMESVKNGTYDYPKYQDESKLNRQEIESVKLES

SEQ ID NO: 88 - protein, 179 aa, Influenza virus A
  influenza A HA2 domain subtype H7 stem domain
GLFGAIAGFIENGWEGLVDGWYGFRHQNAQGEGTAADYKSTQSAIDQITGKLNRLIEKTNQQFELIDNEFTEVEKQIGNLINWTKDSITEVWSYNAELIVAMENQHTIDLADSEMNRLYERVRKQLRENAEEDGTGCFEIFHKCDDDCMASIRNNTYDHSKYREEAMQNRIQIDPVKLS

SEQ ID NO: 89 - protein, 180 aa, Influenza virus A
  influenza A HA2 domain subtype H8 stem domain
GLFGAIAGFIEGGWSGMIDGWYGFHHSNSEGTGMAADQKSTQEAIDKITNKVNNIVDKMNREFEVVNHEFSEVEKRINMINDKIDDQIEDLWAYNAELLVLLENQKTLDEHDSNVKNLFDEVKRRLSANAIDAGNGCFDILHKCDNECMETIKNGTYDHKEYEEEAKLERSKINGVKLEE

SEQ ID NO: 90 - protein, 180 aa, Influenza virus A
  influenza A HA2 domain subtype H9 stem domain
GLFGAIAGFIEGGWPGLVAGWYGFQHSNDQGVGMAADKGSTQKAIDKITSKVNNIIDKMNKQYEVIDHEFNELEARLNMINNKIDDQIQDIWAYNAELLVLLENQKTLDEHDANVNNLYNKVKRALGSNAVEDGNGCFELYHKCDDQCMETIRNGTYDRQKYQEESRLERQKIEGVKLES

SEQ ID NO: 91 - protein, 179 aa, Influenza virus A
  influenza A HA2 domain subtype H10 stem domain
GLFGAIAGFIENGWEGMVDGWYGFRHQNAQGTGQAADYKSTQAAIDQITGKLNRLIEKTNTEFESIESEFSETEHQIGNVINWTKDSITDIWTYNAELLVAMENQHTIDMADSEMLNLYERVRKQLRQNAEEDGKGCFEIYHTCDDSCMESIRNNTYDHSQYREEALLNRLNINPVKLS

SEQ ID NO: 92 - protein, 181 aa, Influenza virus A
  influenza A HA2 domain subtype H11 stem domain
GLFGAIAGFIEGGWPGLINGWYGFQHRDEEGTGIAADKESTQKAIDQITSKVNNIVDRMNTNFESVQHEFSEIEERINQLSKHVDDSVVDIWSYNAQLLVLLENEKTLDLHDSNVRNLHEKVRRMLKDNAKDEGNGCFTFYHKCDNKCIERVRNGTYDHKEFEEESKINRQEIEGVKLDSS

SEQ ID NO: 93 - protein, 180 aa, Influenza virus A
  influenza A HA2 domain subtype H12 stem domain
GLFGAIAGFIEGGWPGLVAGWYGFQHQNAEGTGIAADRDSTQRAIDNMQNKLNNVIDKMNKQFEVVNHEFSEVESRINMINSKIDDQITDIWAYNAELLVLLENQKTLDEHDANVRNLHDRVRRVLRENAIDTGDGCFEILHKCDNNCMDTIRNGTYNHKEYEEESKIERQKVNGVKLEE

SEQ ID NO: 94 - protein, 181 aa, Influenza virus A
  influenza A HA2 domain subtype H13 stem domain
GLFGAIAGFIEGGWPGLINGWYGFQHQNEQGTGIAADKESTQKAIDQITTKINNIIDKMNGNYDSIRGEFNQVEKRINMLADRIDDAVTDIWSYNAKLLVLLENDKTLDMHDANVKNLHEQVRRELKDNAIDEGNGCFELLHKCNDSCMETIRNGTYDHTEYAEESKLKRQEIDGIKLKSE

SEQ ID NO: 95 - protein, 179 aa, Influenza virus A
  influenza A HA2 domain subtype H14 stem domain
GLFGAIAGFIENGWQGLIDGWYGFRHQNAEGTGTAADLKSTQAAIDQINGKLNRLIEKTNEKYHQIEKEFEQVEGRIQDLEKYVEDTKIDLWSYNAELLVALENQHTIDVTDSEMNKLFERVRRQLRENAEDQGNGCFEIFHQCDNNCIESIRNGTYDHNIYRDEAINNRIKINPVTLT

SEQ ID NO: 96 - protein, 179 aa, Influenza virus A
  influenza A HA2 domain subtype H15 stem domain
GLFGAIAGFIENGWEGLIDGWYGFRHQNAQGQGTAADYKSTQAAIDQITGKLNRLIEKTNKQFELIDNEFTEVEQQIGNVINWTRDSLTEIWSYNAELLVAMENQHTIDLADSEMNKLYERVRRQLRENAEEDGTGCFEIFHRCDDQCMESIRNNTYNHTEYRQEALQNRIMINPVKLS

SEQ ID NO: 97 - protein, 181 aa, Influenza virus A
  influenza A HA2 domain subtype H16 stem domain
GLFGAIAGFIEGGWPGLINGWYGFQHQNEQGTGIAADKASTQKAINEITTKINNIIEKMNGNYDSIRGEFNQVEKRINMLADRVDDAVTDIWSYNAKLLVLLENDRTLDLHDANVRNLHDQVKRALKSNAIDEGDGCFNLLHKCNDSCMETIRNGTYNHEDYREESQLKRQEIEGIKLKTE

SEQ ID NO: 98 - protein, 5 aa, Influenza virus A
  influenza A HA2 domain subtype H1 Luminal domain
MGIYQ

SEQ ID NO: 99 - protein, 5 aa, Influenza virus A
  influenza A HA2 domain subtype H2 Luminal domain
MGVYQ

SEQ ID NO: 100 - protein, 5 aa, Influenza virus A
  influenza A HA2 domain subtype H3 Luminal domain
SGYKD

SEQ ID NO: 101 - protein, 5 aa, Influenza virus A
  influenza A HA2 domain subtype H4 Luminal domain
QGYKD

SEQ ID NO: 102 - protein, 5 aa, Influenza virus A
  influenza A HA2 domain subtype H5 Luminal domain
MGVYQ

SEQ ID NO: 103 - protein, 5 aa, Influenza virus A
  influenza A HA2 domain subtype H6 Luminal domain
LGVYQ

SEQ ID NO: 104 - protein, 5 aa, Influenza virus A
  influenza A HA2 domain subtype H7 Luminal domain
SGYKD

SEQ ID NO: 105 - protein, 5 aa, Influenza virus A
  influenza A HA2 domain subtype H8 Luminal domain
NTTYK

SEQ ID NO: 106 - protein, 5 aa, Influenza virus A
  influenza A HA2 domain subtype H9 Luminal domain
EGTYK

SEQ ID NO: 107 - protein, 5 aa, Influenza virus A
  influenza A HA2 domain subtype H10 Luminal domain
SGYKD

SEQ ID NO: 108 - protein, 5 aa, Influenza virus A
  influenza A HA2 domain subtype H11 Luminal domain
GNVYK

SEQ ID NO: 109 - protein, 5 aa, Influenza virus A
  influenza A HA2 domain subtype H12 Luminal domain
NSTYK

SEQ ID NO: 110 - protein, 5 aa, Influenza virus A
  influenza A HA2 domain subtype H13 Luminal domain
DNVYK

SEQ ID NO: 111 - protein, 5 aa, Influenza virus A
  influenza A HA2 domain subtype H14 Luminal domain
MGYKD

SEQ ID NO: 112 - protein, 5 aa, Influenza virus A
  influenza A HA2 domain subtype H15 Luminal domain
SGYKD

SEQ ID NO: 113 - protein, 5 aa, Influenza virus A
  influenza A HA2 domain subtype H16 Luminal domain
DNVYK

SEQ ID NO: 114 - protein, 27 aa, Influenza virus A
  influenza A HA2 domain subtype H1 transmembrane domain
ILAIYSTVASSLVLLVSLGAISFWMCS

SEQ ID NO: 115 - protein, 27 aa, Influenza virus A
  influenza A HA2 domain subtype H2 transmembrane domain
ILAIYATVAGSLSLAIMIAGISLWMCS

SEQ ID NO: 116 - protein, 27 aa, Influenza virus A
  influenza A HA2 domain subtype H3 transmembrane domain
WILWISFAISCFLLCVVLLGFIMWACQ

SEQ ID NO: 117 - protein, 27 aa, Influenza virus A
  influenza A HA2 domain subtype H4 transmembrane domain
IILWISFSISCFLLVALLLAFILWACQ

SEQ ID NO: 118 - protein, 27 aa, Influenza virus A
  influenza A HA2 domain subtype H5 transmembrane domain
ILSIYSTVASSLALAIMIAGLSFWMCS

SEQ ID NO: 119 - protein, 27 aa, Influenza virus A
  influenza A HA2 domain subtype H6 transmembrane domain
ILAIYSTVSSSLVLVGLIIAVGLWMCS

SEQ ID NO: 120 - protein, 27 aa, Influenza virus A
  influenza A HA2 domain subtype H7 transmembrane domain
VILWFSFGASCFLLLAIAMGLVFICVK

SEQ ID NO: 121 - protein, 27 aa, Influenza virus A
  influenza A HA2 domain subtype H8 transmembrane domain
ILSIYSTVAASLCLAILIAGGLILGMQ

SEQ ID NO: 122 - protein, 27 aa, Influenza virus A
  influenza A HA2 domain subtype H9 transmembrane domain
ILTIYSTVASSLVLAMGFAAFLFWAMS

SEQ ID NO: 123 - protein, 27 aa, Influenza virus A
  influenza A HA2 domain subtype H10 transmembrane domain
IILWFSFGESCFVLLAVVMGLVFFCLK

SEQ ID NO: 124 - protein, 27 aa, Influenza virus A
  influenza A HA2 domain subtype H11 transmembrane domain
ILSIYSCIASSLVLAALIMGFMFWACS

SEQ ID NO: 125 - protein, 28 aa, Influenza virus A
  influenza A HA2 domain subtype H12 transmembrane domain
ILSIYSSVASSLVLLLMIIGGFIFGCQN

SEQ ID NO: 126 - protein, 28 aa, Influenza virus A
  influenza A HA2 domain subtype H13 transmembrane domain
ALSIYSCIASSVVLVGLILSFIMWACSS

SEQ ID NO: 127 - protein, 27 aa, Influenza virus A
  influenza A HA2 domain subtype H14 transmembrane domain
IILWISFSMSCFVFVALILGFVLWACQ

SEQ ID NO: 128 - protein, 28 aa, Influenza virus A
  influenza A HA2 domain subtype H15 transmembrane domain
VILWFSFGASCVMLLAIAMGLIFMCVKN

SEQ ID NO: 129 - protein, 27 aa, Influenza virus A
  influenza A HA2 domain subtype H16 transmembrane domain
VLSIYSCIASSIVLVGLILAFIMWACS

SEQ ID NO: 130 - protein, 10 aa, Influenza virus A
  influenza A HA2 domain subtype H1 cytoplasmic domain
NGSLQCRICI

SEQ ID NO: 131 - protein, 10 aa, Influenza virus A
  influenza A HA2 domain subtype H2 cytoplasmic domain
NGSLQCRICI

SEQ ID NO: 132 - protein, 10 aa, Influenza virus A
  influenza A HA2 domain subtype H3 cytoplasmic domain
RGNIRCNICI

SEQ ID NO: 133 - protein, 10 aa, Influenza virus A
  influenza A HA2 domain subtype H4 cytoplasmic domain
NGNIRCQICI

SEQ ID NO: 134 - protein, 10 aa, Influenza virus A
  influenza A HA2 domain subtype H5 cytoplasmic domain
NGSLQCRICI

SEQ ID NO: 135 - protein, 10 aa, Influenza virus A
  influenza A HA2 domain subtype H6 cytoplasmic domain
NGSMQCRICI

SEQ ID NO: 136 - protein, 10 aa, Influenza virus A
  influenza A HA2 domain subtype H7 cytoplasmic domain
NGNMRCTICI

SEQ ID NO: 137 - protein, 10 aa, Influenza virus A
  influenza A HA2 domain subtype H8 cytoplasmic domain
NGSCRCMFCI

SEQ ID NO: 138 - protein, 10 aa, Influenza virus A
  influenza A HA2 domain subtype H9 cytoplasmic domain
NGSCRCNICI

SEQ ID NO: 139 - protein, 10 aa, Influenza virus A
  influenza A HA2 domain subtype H10 cytoplasmic domain
NGNMRCTICI

SEQ ID NO: 140 - protein, 10 aa, Influenza virus A
  influenza A HA2 domain subtype H11 cytoplasmic domain
NGSCRCTICI

SEQ ID NO: 141 - protein, 9 aa, Influenza virus A
  influenza A HA2 domain subtype H12 cytoplasmic domain
GNVRCTFCI

SEQ ID NO: 142 - protein, 9 aa, Influenza virus A
  influenza A HA2 domain subtype H13 cytoplasmic domain
GNCRFNVCI

SEQ ID NO: 143 - protein, 10 aa, Influenza virus A
  influenza A HA2 domain subtype H14 cytoplasmic domain
NGNIRCQICI

SEQ ID NO: 144 - protein, 9 aa, Influenza virus A
  influenza A HA2 domain subtype H15 cytoplasmic domain
GNLRCTICI

SEQ ID NO: 145 - protein, 10 aa, Influenza virus A
  influenza A HA2 domain subtype H16 cytoplasmic domain
NGSCRFNVCI

SEQ ID NO: 146 - protein, 23 aa, Artificial Sequence
  sequence of HA1 N-terminal stem segment
  VARIANT 1: Xaa = Tyr or His
  VARIANT 2: Xaa = His, Leu or Gln
  VARIANT 3.....20: Xaa = any amino acid
  VARIANT 21: Xaa = any amino acid or absent
  VARIANT 21: Xaa = any amino acid or absent
  VARIANT 23: Xaa = His, Ser, Gln, Thr or Asn
XXXXXXXXXXXXXXXXXXXXXXX

SEQ ID NO: 147 - protein, 2 aa, Artificial Sequence
  sequence of HA1 c-terminal stem segment
  VARIANT 1: Xaa = Thr, Ser, Asn, Asp, Pro or Lys
  VARIANT 2: Xaa = Leu, Met, Lys or Arg
XX

SEQ ID NO: 148 - protein, 4 aa, Artificial Sequence
  sequence of HA2 domain
  VARIANT 1: Xaa = Val or Ile
  VARIANT 1: Xaa = Asp, Asn or Ala
XXGW

SEQ ID NO: 149 - protein, 19 aa, Artificial Sequence
  sequence of HA2 domain
  VARIANT 1: Xaa = Lys, Gln, Arg, Leu or Tyr
  VARIANT 2, 3, 6, 10, 13, 17: Xaa = any amino acid
  VARIANT 11: Xaa = Ile, Val or Met
  VARIANT 12: Xaa = Thr, Gln or Asn
  VARIANT 15: Xaa = Val or Leu
  VARIANT 18: Xaa = Val, Ile or Leu
  VARIANT 19: Xaa = Val or Ile
XXXTQXAIDXXXXKXNXXX

SEQ ID NO: 150 - protein, 15 aa, Influenza virus B
  Signal peptide of Influenza B HA construct variant Arg50-Ser277
MKAIIVILMVVTSNA

SEQ ID NO: 151 - protein, 15 aa, Influenza virus B
  Signal peptide of Influenza B HA construct variant Ala66-Trp271
MKAIIVILMVVTSNA

SEQ ID NO: 152 - protein, 15 aa, Influenza virus B
  Signal peptide of Influenza B HA construct variant Lys80-Ser277
MKAIIVILMVVTSNA

SEQ ID NO: 153 - protein, 15 aa, Influenza virus B
  Signal peptide of Influenza B HA construct variant Arg80-Ser277
MKAIIVILMVVTSNA

SEQ ID NO: 154 - protein, 50 aa, Influenza virus B
  HA1 N-terminal Stem Segment of Influenza B HA construct variant Arg50-Ser277
DRICTGITSSNSPHVVKTATQGEVNVTGVIPLTTTPTKSHFANLKGTETR

SEQ ID NO: 155 - protein, 66 aa, Influenza virus B
  HA1 N-terminal Stem Segment of Influenza B HA construct variant Ala66-Trp271
DRICTGITSSNSPHVVKTATQGEVNVTGVIPLTTTPTKSHFANLKGTETRGKLCPKCLNCTDLDVA

SEQ ID NO: 156 - protein, 80 aa, Influenza virus B
  HA1 N-terminal Stem Segment of Influenza B HA construct variant Lys80-Ser277
DRICTGITSSNSPHVVKTATQGEVNVTGVIPLTTTPTKSHFANLKGTETRGKLCPKCLNCTDLDVALGRPKCTGKIPSAK

SEQ ID NO: 157 - protein, 80 aa, Influenza virus B
  HA1 N-terminal Stem Segment of Influenza B HA construct variant Arg80-Ser277
DRICTGITSSNSPHVVKTATQGEVNVTGVIPLTTTPTKSHFANLKGTETRGKLCPKCLNCTDLDVALGRPKCTGKIPSAR

SEQ ID NO: 158 - protein, 68 aa, Influenza virus B
  HA1 C-terminal Stem Segment of Influenza B HA construct variant Arg50-Ser277
SKVIKGSLPLIGEADCLHEKYGGLNKSKPYYTGEHAKAIGNCPIWVKTPLKLANGTKYRPPAKLLKER

SEQ ID NO: 159 - protein, 74 aa, Influenza virus B
  HA1 C-terminal Stem Segment of Influenza B HA construct variant Ala66-Trp271
WCASGRSKVIKGSLPLIGEADCLHEKYGGLNKSKPYYTGEHAKAIGNCPIWVKTPLKLANGTKYRPPAKLLKER

SEQ ID NO: 160 - protein, 223 aa, Influenza virus B
  HA2 Domain of Influenza B HA construct variant Arg50-Ser277 and other variants listed in Table 3
GFFGAIAGFLEGGWEGMIAGWHGYTSHGAHGVAVAADLKSTQEAINKITKNLNSLSELEVKNLQRLSGAMDELHNEILELDEKVDDLRADTISSQIELAVLLSNEGIINSEDEHLLALERKLKKMLGPSAVEIGNGCFETKHKCNQTCLDRIAAGTFDAGEFSLPTFDSLNITAASLNDDGLDNHTILLYYSTAASSLAVTLMIAIFVVYMVSRDNVSCSICL

SEQ ID NO: 161 - protein, 179 aa, Influenza virus B
  Stem domain of Influenza B HA2 domain subtype HA2
GFFGAIAGFLEGGWEGMIAGWHGYTSHGAHGVAVAADLKSTQEAINKITKNLNSLSELEVKNLQRLSGAMDELHNEILELDEKVDDLRADTISSQIELAVLLSNEGIINSEDEHLLALERKLKKMLGPSAVEIGNGCFETKHKCNQTCLDRIAAGTFDAGEFSLPTFDSLNITAASLND

SEQ ID NO: 162 - protein, 5 aa, Influenza virus B
  luminal domain of Influenza B HA2 domain subtype HA2
DGLDN

SEQ ID NO: 163 - protein, 28 aa, Influenza virus B
  transmembrane domain of Influenza B HA2 domain subtype HA2
HTILLYYSTAASSLAVTLMIAIFVVYMV

SEQ ID NO: 164 - protein, 11 aa, Influenza virus B
  cytoplasmic domain of Influenza B HA2 domain subtype HA2
SRDNVSCSICL

SEQ ID NO: 165 - protein, 23 aa, Artificial Sequence
  turn loop linker sequence
ITPNGSIPNDKPFQNVNKITYGA

SEQ ID NO: 166 - protein, 6 aa, Artificial Sequence
  His tag
HHHHHH

SEQ ID NO: 167 - protein, 29 aa, Artificial Sequence
  example of a foldon domain
GSGYIPEAPRDGQAYVRKDGEWVLLSTFL

SEQ ID NO: 168 - protein, 7 aa, Artificial Sequence
  thrombin cleavage site
LVPRGSP

SEQ ID NO: 169-176 - skipped (8 entries)

SEQ ID NO: 177 - protein, 41 aa, Influenza virus A
  N-terminal stem segment of Influenza A HA subtype H1(no Cys) Short Stem Domain sequence
DTICIGYHANNSTDTVDTVLEKNVTVTHSVNLLEDSHNGKL

SEQ ID NO: 178 - protein, 41 aa, Influenza virus A; identical to SEQ ID NO: 177
  N-terminal stem segment of Influenza A HA subtype H1(no Cys-delta 1) Short Stem Domain sequence

SEQ ID NO: 179 - protein, 40 aa, Influenza virus A
  N-terminal stem segment of Influenza A HA subtype H1(no Cys-delta 3) Short Stem Domain sequence
DTICIGYHANNSTDTVDTVLEKNVTVTHSVNLLEDSHNGK

SEQ ID NO: 180 - protein, 41 aa, Influenza virus A
  N-terminal stem segment of Influenza A HA subtype H2(no Cys) Short Stem Domain sequence
DQICIGYHSNNSTEKVDTILERNVTVTHAQNILEKTHNGKL

SEQ ID NO: 181 - protein, 41 aa, Influenza virus A; identical to SEQ ID NO: 180
  N-terminal stem segment of Influenza A HA subtype H2(no Cys-delta 1) Short Stem Domain sequence

SEQ ID NO: 182 - protein, 40 aa, Influenza virus A
  N-terminal stem segment of Influenza A HA subtype H2(no Cys-delta 3) Short Stem Domain sequence
DQICIGYHSNNSTEKVDTILERNVTVTHAQNILEKTHNGK

SEQ ID NO: 183 - protein, 51 aa, Influenza virus A
  N-terminal stem segment of Influenza A HA subtype H3(no Cys) Short Stem Domain sequence
QDLPGNDNSTATLCLGHHAVPNGTLVKTITDDQIEVTNATELVQSSSTGKI

SEQ ID NO: 184 - protein, 51 aa, Influenza virus A; identical to SEQ ID NO: 183
  N-terminal stem segment of Influenza A HA subtype H3(no Cys-delta 1) Short Stem Domain sequence

SEQ ID NO: 185 - protein, 50 aa, Influenza virus A
  N-terminal stem segment of Influenza A HA subtype H3(no Cys-delta 3) Short Stem Domain sequence
QDLPGNDNSTATLCLGHHAVPNGTLVKTITDDQIEVTNATELVQSSSTGK

SEQ ID NO: 186 - protein, 47 aa, Influenza virus A
  N-terminal stem segment of Influenza A HA subtype H4(no Cys) Short Stem Domain sequence
QNYTGNPVICMGHHAVANGTMVKTLADDQVEVVTAQELVESQNLPEL

SEQ ID NO: 187 - protein, 47 aa, Influenza virus A; identical to SEQ ID NO: 186
  N-terminal stem segment of Influenza A HA subtype H4(no Cys-delta 1) Short Stem Domain sequence

SEQ ID NO: 188 - protein, 46 aa, Influenza virus A
  N-terminal stem segment of Influenza A HA subtype H4(no Cys-delta 3) Short Stem Domain sequence
QNYTGNPVICMGHHAVANGTMVKTLADDQVEVVTAQELVESQNLPE

SEQ ID NO: 189 - protein, 41 aa, Influenza virus A
  N-terminal stem segment of Influenza A HA subtype H5(no Cys) Short Stem Domain sequence
DQICIGYHANKSTKQVDTIMEKNVTVTHAQDILERTHNGKL

SEQ ID NO: 190 - protein, 41 aa, Influenza virus A; identical to SEQ ID NO: 189
  N-terminal stem segment of Influenza A HA subtype H5(no Cys-delta 1) Short Stem Domain sequence

SEQ ID NO: 191 - protein, 40 aa, Influenza virus A
  N-terminal stem segment of Influenza A HA subtype H5(no Cys-delta 3) Short Stem Domain sequence
DQICIGYHANKSTKQVDTIMEKNVTVTHAQDILERTHNGK

SEQ ID NO: 192 - protein, 41 aa, Influenza virus A
  N-terminal stem segment of Influenza A HA subtype H6(no Cys) Short Stem Domain sequence
DKICIGYHANNSTTQIDTILEKNVTVTHSVELLENQKEERF

SEQ ID NO: 193 - protein, 41 aa, Influenza virus A; identical to SEQ ID NO: 192
  N-terminal stem segment of Influenza A HA subtype H6(no Cys-delta 1) Short Stem Domain sequence

SEQ ID NO: 194 - protein, 40 aa, Influenza virus A
  N-terminal stem segment of Influenza A HA subtype H6(no Cys-delta 3) Short Stem Domain sequence
DKICIGYHANNSTTQIDTILEKNVTVTHSVELLENQKEER

SEQ ID NO: 195 - protein, 41 aa, Influenza virus A
  N-terminal stem segment of Influenza A HA subtype H7(no Cys) Short Stem Domain sequence
DKICLGHHAVSNGTKVNTLTERGVEVVNATETVERTNIPKI

SEQ ID NO: 196 - protein, 41 aa, Influenza virus A; identical to SEQ ID NO: 195
  N-terminal stem segment of Influenza A HA subtype H7(no Cys-delta 1) Short Stem Domain sequence

SEQ ID NO: 197 - protein, 40 aa, Influenza virus A
  N-terminal stem segment of Influenza A HA subtype H7(no Cys-delta 3) Short Stem Domain sequence
DKICLGHHAVSNGTKVNTLTERGVEVVNATETVERTNIPK

SEQ ID NO: 198 - protein, 41 aa, Influenza virus A
  N-terminal stem segment of Influenza A HA subtype H8(no Cys) Short Stem Domain sequence
DRICIGYQSNNSTDTVNTLIEQNVPVTQTMELVETEKHPAY

SEQ ID NO: 199 - protein, 41 aa, Influenza virus A; identical to SEQ ID NO: 198
  N-terminal stem segment of Influenza A HA subtype H8(no Cys-delta 1) Short Stem Domain sequence

SEQ ID NO: 200 - protein, 40 aa, Influenza virus A
  N-terminal stem segment of Influenza A HA subtype H8(no Cys-delta 3) Short Stem Domain sequence
DRICIGYQSNNSTDTVNTLIEQNVPVTQTMELVETEKHPA

SEQ ID NO: 201 - protein, 41 aa, Influenza virus A
  N-terminal stem segment of Influenza A HA subtype H9(no Cys) Short Stem Domain sequence
DKICIGYQSTNSTETVDTLTESNVPVTHTKELLHTEHNGML

SEQ ID NO: 202 - protein, 41 aa, Influenza virus A; identical to SEQ ID NO: 201
  N-terminal stem segment of Influenza A HA subtype H9(no Cys-delta 1) Short Stem Domain sequence

SEQ ID NO: 203 - protein, 40 aa, Influenza virus A
  N-terminal stem segment of Influenza A HA subtype H9(no Cys-delta 3) Short Stem Domain sequence
DKICIGYQSTNSTETVDTLTESNVPVTHTKELLHTEHNGM

SEQ ID NO: 204 - protein, 42 aa, Influenza virus A
  N-terminal stem segment of Influenza A HA subtype H10(no Cys) Short Stem Domain sequence
LDRICLGHHAVANGTIVKTLTNEQEEVTNATETVESTNLNKL

SEQ ID NO: 205 - protein, 42 aa, Influenza virus A; identical to SEQ ID NO: 204
  N-terminal stem segment of Influenza A HA subtype H10(no Cys-delta 1) Short Stem Domain sequence

SEQ ID NO: 206 - protein, 41 aa, Influenza virus A
  N-terminal stem segment of Influenza A HA subtype H10(no Cys-delta 3) Short Stem Domain sequence
LDRICLGHHAVANGTIVKTLTNEQEEVTNATETVESTNLNK

SEQ ID NO: 207 - protein, 41 aa, Influenza virus A
  N-terminal stem segment of Influenza A HA subtype H11(no Cys) Short Stem Domain sequence
DEICIGYLSNNSTDKVDTIIENNVTVTSSVELVETEHTGSF

SEQ ID NO: 208 - protein, 41 aa, Influenza virus A; identical to SEQ ID NO: 207
  N-terminal stem segment of Influenza A HA subtype H11(no Cys-delta 1) Short Stem Domain sequence

SEQ ID NO: 209 - protein, 40 aa, Influenza virus A
  N-terminal stem segment of Influenza A HA subtype H11(no Cys-delta 3) Short Stem Domain sequence
DEICIGYLSNNSTDKVDTIIENNVTVTSSVELVETEHTGS

SEQ ID NO: 210 - protein, 41 aa, Influenza virus A
  N-terminal stem segment of Influenza A HA subtype H12(no Cys) Short Stem Domain sequence
DKICIGYQTNNSTETVNTLSEQNVPVTQVEELVHRGIDPIL

SEQ ID NO: 211 - protein, 41 aa, Influenza virus A; identical to SEQ ID NO: 210
  N-terminal stem segment of Influenza A HA subtype H12(no Cys-delta 1) Short Stem Domain sequence

SEQ ID NO: 212 - protein, 40 aa, Influenza virus A
  N-terminal stem segment of Influenza A HA subtype H12(no Cys-delta 3) Short Stem Domain sequence
DKICIGYQTNNSTETVNTLSEQNVPVTQVEELVHRGIDPI

SEQ ID NO: 213 - protein, 41 aa, Influenza virus A
  N-terminal stem segment of Influenza A HA subtype H13(no Cys) Short Stem Domain sequence
DRICVGYLSTNSSERVDTLLENGVPVTSSIDLIETNHTGTY

SEQ ID NO: 214 - protein, 41 aa, Influenza virus A; identical to SEQ ID NO: 213
  N-terminal stem segment of Influenza A HA subtype H13(no Cys-delta 1) Short Stem Domain sequence

SEQ ID NO: 215 - protein, 40 aa, Influenza virus A
  N-terminal stem segment of Influenza A HA subtype H13(no Cys-delta 3) Short Stem Domain sequence
DRICVGYLSTNSSERVDTLLENGVPVTSSIDLIETNHTGT

SEQ ID NO: 216 - protein, 50 aa, Influenza virus A
  N-terminal stem segment of Influenza A HA subtype H14(no Cys) Short Stem Domain sequence
QITNGTTGNPIICLGHHAVENGTSVKTLTDNHVEVVSAKELVETNHTDEL

SEQ ID NO: 217 - protein, 50 aa, Influenza virus A; identical to SEQ ID NO: 216
  N-terminal stem segment of Influenza A HA subtype H14(no Cys-delta 1) Short Stem Domain sequence

SEQ ID NO: 218 - protein, 49 aa, Influenza virus A
  N-terminal stem segment of Influenza A HA subtype H14(no Cys-delta 3) Short Stem Domain sequence
QITNGTTGNPIICLGHHAVENGTSVKTLTDNHVEVVSAKELVETNHTDE

SEQ ID NO: 219 - protein, 41 aa, Influenza virus A
  N-terminal stem segment of Influenza A HA subtype H15(no Cys) Short Stem Domain sequence
DKICLGHHAVANGTKVNTLTERGVEVVNATETVEITGIDKV

SEQ ID NO: 220 - protein, 41 aa, Influenza virus A; identical to SEQ ID NO: 219
  N-terminal stem segment of Influenza A HA subtype H15(no Cys-delta 1) Short Stem Domain sequence

SEQ ID NO: 221 - protein, 40 aa, Influenza virus A
  N-terminal stem segment of Influenza A HA subtype H15(no Cys-delta 3) Short Stem Domain sequence
DKICLGHHAVANGTKVNTLTERGVEVVNATETVEITGIDK

SEQ ID NO: 222 - protein, 41 aa, Influenza virus A
  N-terminal stem segment of Influenza A HA subtype H16(no Cys) Short Stem Domain sequence
DKICIGYLSNNSSDTVDTLTENGVPVTSSVDLVETNHTGTY

SEQ ID NO: 223 - protein, 41 aa, Influenza virus A; identical to SEQ ID NO: 222
  N-terminal stem segment of Influenza A HA subtype H16(no Cys-delta 1) Short Stem Domain sequence

SEQ ID NO: 224 - protein, 40 aa, Influenza virus A
  N-terminal stem segment of Influenza A HA subtype H16(no Cys-delta 3) Short Stem Domain sequence
DKICIGYLSNNSSDTVDTLTENGVPVTSSVDLVETNHTGT

SEQ ID NO: 225 - skipped

SEQ ID NO: 226 - protein, 52 aa, Influenza virus A
  C-terminal stem segment of Influenza A HA subtype H1(no Cys)
NTKCQTPLGAINSSLPYQNIHPVTIGECPKYVRSAKLRMVTGLRNNPSIQSR

SEQ ID NO: 227 - protein, 51 aa, Influenza virus A
  C-terminal stem segment of Influenza A HA subtype H1(no Cys-delta 1)
TKCQTPLGAINSSLPYQNIHPVTIGECPKYVRSAKLRMVTGLRNNPSIQSR

SEQ ID NO: 228 - protein, 50 aa, Influenza virus A
  C-terminal stem segment of Influenza A HA subtype H1(no Cys-delta 3)
KCQTPLGAINSSLPYQNIHPVTIGECPKYVRSAKLRMVTGLRNNPSIQSR

SEQ ID NO: 229 - protein, 52 aa, Influenza virus A
  C-terminal stem segment of Influenza A HA subtype H2(no Cys)
ETKCQTPLGAINTTLPFHNVHPLTIGECPKYVKSERLVLATGLRNVPQIESR

SEQ ID NO: 230 - protein, 51 aa, Influenza virus A
  C-terminal stem segment of Influenza A HA subtype H2(no Cys-delta 1)
TKCQTPLGAINTTLPFHNVHPLTIGECPKYVKSERLVLATGLRNVPQIESR

SEQ ID NO: 231 - protein, 50 aa, Influenza virus A
  C-terminal stem segment of Influenza A HA subtype H2(no Cys-delta 3)
KCQTPLGAINTTLPFHNVHPLTIGECPKYVKSERLVLATGLRNVPQIESR

SEQ ID NO: 232 - protein, 52 aa, Influenza virus A
  C-terminal stem segment of Influenza A HA subtype H3(no Cys)
ISECITPNGSIPNDKPFQNVNKITYGACPKYVKQNTLKLATGMRNVPEKQTR

SEQ ID NO: 233 - protein, 51 aa, Influenza virus A
  C-terminal stem segment of Influenza A HA subtype H3(no Cys-delta 1)
SECITPNGSIPNDKPFQNVNKITYGACPKYVKQNTLKLATGMRNVPEKQTR

SEQ ID NO: 234 - protein, 50 aa, Influenza virus A
  C-terminal stem segment of Influenza A HA subtype H3(no Cys-delta 3)
ECITPNGSIPNDKPFQNVNKITYGACPKYVKQNTLKLATGMRNVPEKQTR

SEQ ID NO: 235 - protein, 52 aa, Influenza virus A
  C-terminal stem segment of Influenza A HA subtype H4(no Cys)
VSKCHTDKGSLSTTKPFQNISRIAVGDCPRYVKQGSLKLATGMRNIPEKASR

SEQ ID NO: 236 - protein, 51 aa, Influenza virus A
  C-terminal stem segment of Influenza A HA subtype H4(no Cys-delta 1)
SKCHTDKGSLSTTKPFQNISRIAVGDCPRYVKQGSLKLATGMRNIPEKASR

SEQ ID NO: 237 - protein, 50 aa, Influenza virus A
  C-terminal stem segment of Influenza A HA subtype H4(no Cys-delta 3)
KCHTDKGSLSTTKPFQNISRIAVGDCPRYVKQGSLKLATGMRNIPEKASR

SEQ ID NO: 238 - protein, 52 aa, Influenza virus A
  C-terminal stem segment of Influenza A HA subtype H5(no Cys)
DTKCQTPVGEINSSMPFHNIHPHTIGECPKYVKSDRLVLATGLRNVPQRKKR

SEQ ID NO: 239 - protein, 51 aa, Influenza virus A
  C-terminal stem segment of Influenza A HA subtype H5(no Cys-delta 1)
TKCQTPVGEINSSMPFHNIHPHTIGECPKYVKSDRLVLATGLRNVPQRKKR

SEQ ID NO: 240 - protein, 50 aa, Influenza virus A
  C-terminal stem segment of Influenza A HA subtype H5(no Cys-delta 3)
KCQTPVGEINSSMPFHNIHPHTIGECPKYVKSDRLVLATGLRNVPQRKKR

SEQ ID NO: 241 - protein, 52 aa, Influenza virus A
  C-terminal stem segment of Influenza A HA subtype H6(no Cys)
DATCQTVAGVLRTNKTFQNVSPLWIGECPKYVKSESLRLATGLRNVPQIETR

SEQ ID NO: 242 - protein, 51 aa, Influenza virus A
  C-terminal stem segment of Influenza A HA subtype H6(no Cys-delta 1)
ATCQTVAGVLRTNKTFQNVSPLWIGECPKYVKSESLRLATGLRNVPQIETR

SEQ ID NO: 243 - protein, 50 aa, Influenza virus A
  C-terminal stem segment of Influenza A HA subtype H6(no Cys-delta 3)
TCQTVAGVLRTNKTFQNVSPLWIGECPKYVKSESLRLATGLRNVPQIETR

SEQ ID NO: 244 - protein, 56 aa, Influenza virus A
  C-terminal stem segment of Influenza A HA subtype H7(no Cys)
EGECYHSGGTITSRLPFQNINSRAVGKCPRYVKQESLLLATGMKNVPEPSKKRKKR

SEQ ID NO: 245 - protein, 55 aa, Influenza virus A
  C-terminal stem segment of Influenza A HA subtype H7(no Cys-delta 1)
GECYHSGGTITSRLPFQNINSRAVGKCPRYVKQESLLLATGMKNVPEPSKKRKKR

SEQ ID NO: 246 - protein, 54 aa, Influenza virus A
  C-terminal stem segment of Influenza A HA subtype H7(no Cys-delta 3)
ECYHSGGTITSRLPFQNINSRAVGKCPRYVKQESLLLATGMKNVPEPSKKRKKR

SEQ ID NO: 247 - protein, 52 aa, Influenza virus A
  C-terminal stem segment of Influenza A HA subtype H8(no Cys)
NTKCQTYAGAINSSKPFQNASRHYMGECPKYVKKASLRLAVGLRNTPSVEPR

SEQ ID NO: 248 - protein, 51 aa, Influenza virus A
  C-terminal stem segment of Influenza A HA subtype H8(no Cys-delta 1)
TKCQTYAGAINSSKPFQNASRHYMGECPKYVKKASLRLAVGLRNTPSVEPR

SEQ ID NO: 249 - protein, 50 aa, Influenza virus A
  C-terminal stem segment of Influenza A HA subtype H8(no Cys-delta 3)
KCQTYAGAINSSKPFQNASRHYMGECPKYVKKASLRLAVGLRNTPSVEPR

SEQ ID NO: 250 - protein, 52 aa, Influenza virus A
  C-terminal stem segment of Influenza A HA subtype H9(no Cys)
VVQCQTEKGGLNTTLPFHNISKYAFGNCPKYVGVKSLKLPVGLRNVPAVSSR

SEQ ID NO: 251 - protein, 51 aa, Influenza virus A
  C-terminal stem segment of Influenza A HA subtype H9(no Cys-delta 1)
VQCQTEKGGLNTTLPFHNISKYAFGNCPKYVGVKSLKLPVGLRNVPAVSSR

SEQ ID NO: 252 - protein, 50 aa, Influenza virus A
  C-terminal stem segment of Influenza A HA subtype H9(no Cys-delta 3)
QCQTEKGGLNTTLPFHNISKYAFGNCPKYVGVKSLKLPVGLRNVPAVSSR

SEQ ID NO: 253 - protein, 53 aa, Influenza virus A
  C-terminal stem segment of Influenza A HA subtype H10(no Cys)
ESKCFWRGGSINTKLPFQNLSPRTVGQCPKYVNQRSLLLATGMRNVPEVVQGR

SEQ ID NO: 254 - protein, 52 aa, Influenza virus A
  C-terminal stem segment of Influenza A HA subtype H10(no Cys-delta 1)
SKCFWRGGSINTKLPFQNLSPRTVGQCPKYVNQRSLLLATGMRNVPEVVQGR

SEQ ID NO: 255 - protein, 51 aa, Influenza virus A
  C-terminal stem segment of Influenza A HA subtype H10(no Cys-delta 3)
KCFWRGGSINTKLPFQNLSPRTVGQCPKYVNQRSLLLATGMRNVPEVVQGR

SEQ ID NO: 256 - protein, 52 aa, Influenza virus A
  C-terminal stem segment of Influenza A HA subtype H11(no Cys)
STKCQTEIGGINTNKSFHNVHRNTIGDCPKYVNVKSLKLATGPRNVPAIASR

SEQ ID NO: 257 - protein, 51 aa, Influenza virus A
  C-terminal stem segment of Influenza A HA subtype H11(no Cys-delta 1)
TKCQTEIGGINTNKSFHNVHRNTIGDCPKYVNVKSLKLATGPRNVPAIASR

SEQ ID NO: 258 - protein, 50 aa, Influenza virus A
  C-terminal stem segment of Influenza A HA subtype H11(no Cys-delta 3)
KCQTEIGGINTNKSFHNVHRNTIGDCPKYVNVKSLKLATGPRNVPAIASR

SEQ ID NO: 259 - protein, 52 aa, Influenza virus A
  C-terminal stem segment of Influenza A HA subtype H12(no Cys)
VTECQLNEGVMNTSKPFQNTSKHYIGKCPKYIPSGSLKLAIGLRNVPQVQDR

SEQ ID NO: 260 - protein, 51 aa, Influenza virus A
  C-terminal stem segment of Influenza A HA subtype H12(no Cys-delta 1)
TECQLNEGVMNTSKPFQNTSKHYIGKCPKYIPSGSLKLAIGLRNVPQVQDR

SEQ ID NO: 261 - protein, 50 aa, Influenza virus A
  C-terminal stem segment of Influenza A HA subtype H12(no Cys-delta 3)
ECQLNEGVMNTSKPFQNTSKHYIGKCPKYIPSGSLKLAIGLRNVPQVQDR

SEQ ID NO: 262 - protein, 52 aa, Influenza virus A
  C-terminal stem segment of Influenza A HA subtype H13(no Cys)
NTKCQTSVGGINTNRTFQNIDKNALGDCPKYIKSGQLKLATGLRNVPAISNR

SEQ ID NO: 263 - protein, 51 aa, Influenza virus A
  C-terminal stem segment of Influenza A HA subtype H13(no Cys-delta 1)
TKCQTSVGGINTNRTFQNIDKNALGDCPKYIKSGQLKLATGLRNVPAISNR

SEQ ID NO: 264 - protein, 50 aa, Influenza virus A
  C-terminal stem segment of Influenza A HA subtype H13(no Cys-delta 3)
KCQTSVGGINTNRTFQNIDKNALGDCPKYIKSGQLKLATGLRNVPAISNR

SEQ ID NO: 265 - protein, 52 aa, Influenza virus A
  C-terminal stem segment of Influenza A HA subtype H14(no Cys)
TSPCLTDKGSIQSDKPFQNVSRIAIGNCPKYVKQGSLMLATGMRNIPGKQAK

SEQ ID NO: 266 - protein, 51 aa, Influenza virus A
  C-terminal stem segment of Influenza A HA subtype H14(no Cys-delta 1)
SPCLTDKGSIQSDKPFQNVSRIAIGNCPKYVKQGSLMLATGMRNIPGKQAK

SEQ ID NO: 267 - protein, 50 aa, Influenza virus A
  C-terminal stem segment of Influenza A HA subtype H14(no Cys-delta 3)
PCLTDKGSIQSDKPFQNVSRIAIGNCPKYVKQGSLMLATGMRNIPGKQAK

SEQ ID NO: 268 - protein, 53 aa, Influenza virus A
  C-terminal stem segment of Influenza A HA subtype H15(no Cys)
EGECFYSGGTINSPLPFQNIDSRAVGKCPRYVKQSSLPLALGMKNVPEKIRTR

SEQ ID NO: 269 - protein, 52 aa, Influenza virus A
  C-terminal stem segment of Influenza A HA subtype H15(no Cys-delta 1)
GECFYSGGTINSPLPFQNIDSRAVGKCPRYVKQSSLPLALGMKNVPEKIRTR

SEQ ID NO: 270 - protein, 51 aa, Influenza virus A
  C-terminal stem segment of Influenza A HA subtype H15(no Cys-delta 3)
ECFYSGGTINSPLPFQNIDSRAVGKCPRYVKQSSLPLALGMKNVPEKIRTR

SEQ ID NO: 271 - protein, 52 aa, Influenza virus A
  C-terminal stem segment of Influenza A HA subtype H16(no Cys)
NTKCQTSLGGINTNKTFQNIERNALGDCPKYIKSGQLKLATGLRNVPSIGER

SEQ ID NO: 272 - protein, 51 aa, Influenza virus A
  C-terminal stem segment of Influenza A HA subtype H16(no Cys-delta 1)
TKCQTSLGGINTNKTFQNIERNALGDCPKYIKSGQLKLATGLRNVPSIGER

SEQ ID NO: 273 - protein, 50 aa, Influenza virus A
  C-terminal stem segment of Influenza A HA subtype H16(no Cys-delta 3)
KCQTSLGGINTNKTFQNIERNALGDCPKYIKSGQLKLATGLRNVPSIGER

SEQ ID NO: 274-307 - skipped (34 entries)

SEQ ID NO: 308 - protein, 44 aa, Influenza virus A
  N-terminal stem segment of Influenza A HA subtype H3(HK68-CON-A)
STATLCLGHHAVPNGTLVKTITDDQIEVTNATELVQSSSTGKIC

SEQ ID NO: 309 - protein, 24 aa, Influenza virus A
  C-terminal stem segment of Influenza A HA subtype H3(HK68-CON-B)
CKYVKQNTLKLATGMRNVPEKQTR

SEQ ID NO: 310 - protein, 97 aa, Influenza virus A
  N-terminal stem segment of Influenza A HA subtype H3(HK68-CON-C)
QDLPGNDNSTATLCLGHHAVPNGTLVKTITDDQIEVTNATELVQSSSTGKICNNPHRILDGIDCTLIDALLGDPHCDVFQNETWDLFVERSKAFSNC

SEQ ID NO: 311 - protein, 74 aa, Influenza virus A
  C-terminal stem segment of Influenza A HA subtype H3(HK68-CON-C)
APRGYFKMRTGKSSIMSSDAPIDTCISECITPNGSIPNDKPFQNVNKITYGACPKYVKQNTLKLATGMRNVPEK

SEQ ID NO: 312 - protein, 46 aa, Influenza virus A
  N-terminal stem segment of Influenza A HA subtype H1(HK68-CON-A)
DTICIGYHANNSTDTVDTVLEKNVTVTHSVNLLEDSHNGKLCRLKC

SEQ ID NO: 313 - protein, 52 aa, Influenza virus A
  C-terminal stem segment of Influenza A HA subtype H1(HK68-CON-A)
CKCQTPLGAINSSLPYQNIHPVTIGECPKYVRSAKLRMVTGLRNNPSIQSRG

SEQ ID NO: 314 - protein, 23 aa, Influenza virus A
  C-terminal stem segment of Influenza A HA subtype H1(HK68-CON-B)
CVRSAKLRMVTGLRNNPSIQSRG

SEQ ID NO: 315 - protein, 94 aa, Influenza virus A
  N-terminal stem segment of Influenza A HA subtype H1(HK68-CON-C)
DTICIGYHANNSTDTVDTVLEKNVTVTHSVNLLEDSHNGKLCRLKGIAPLQLGKCNIAGWLLGNPECDPLLPVRSWSYIVETPNSENGICYPGC

SEQ ID NO: 316 - protein, 75 aa, Influenza virus A
  C-terminal stem segment of Influenza A HA subtype H1(HK68-CON-C)
AFALSRGFGSGIITSNASMHECNTKCQTPLGAINSSLPYQNIHPVTIGECPKYVRSAKLRMVTGLRNNPSIQSRG

SEQ ID NO: 317-349 - skipped (33 entries)

SEQ ID NO: 350 - protein, 25 aa, Influenza virus A
  C-terminal short stem segment of Influenza A HA subtype H1
CPKYVRSAKLRMVTGLRNNPSIQSR

SEQ ID NO: 351 - protein, 25 aa, Influenza virus A
  C-terminal short stem segment of Influenza A HA subtype H2
CPKYVKSERLVLATGLRNVPQIESR

SEQ ID NO: 352 - protein, 25 aa, Influenza virus A
  C-terminal short stem segment of Influenza A HA subtype H3
CPKYVKQNTLKLATGMRNVPEKQTR

SEQ ID NO: 353 - protein, 25 aa, Influenza virus A
  C-terminal short stem segment of Influenza A HA subtype H4
CPRYVKQGSLKLATGMRNIPEKASR

SEQ ID NO: 354 - protein, 25 aa, Influenza virus A
  C-terminal short stem segment of Influenza A HA subtype H5
CPKYVKSDRLVLATGLRNVPQRKKR

SEQ ID NO: 355 - protein, 25 aa, Influenza virus A
  C-terminal short stem segment of Influenza A HA subtype H6
CPKYVKSESLRLATGLRNVPQIETR

SEQ ID NO: 356 - protein, 29 aa, Influenza virus A
  C-terminal short stem segment of Influenza A HA subtype H7
CPRYVKQESLLLATGMKNVPEPSKKRKKR

SEQ ID NO: 357 - protein, 25 aa, Influenza virus A
  C-terminal short stem segment of Influenza A HA subtype H8
CPKYVKKASLRLAVGLRNTPSVEPR

SEQ ID NO: 358 - protein, 25 aa, Influenza virus A
  C-terminal short stem segment of Influenza A HA subtype H9
CPKYVGVKSLKLPVGLRNVPAVSSR

SEQ ID NO: 359 - protein, 26 aa, Influenza virus A
  C-terminal short stem segment of Influenza A HA subtype H10
CPKYVNQRSLLLATGMRNVPEVVQGR

SEQ ID NO: 360 - protein, 25 aa, Influenza virus A
  C-terminal short stem segment of Influenza A HA subtype H11
CPKYVNVKSLKLATGPRNVPAIASR

SEQ ID NO: 361 - protein, 25 aa, Influenza virus A
  C-terminal short stem segment of Influenza A HA subtype H12
CPKYIPSGSLKLAIGLRNVPQVQDR

SEQ ID NO: 362 - protein, 25 aa, Influenza virus A
  C-terminal short stem segment of Influenza A HA subtype H13
CPKYIKSGQLKLATGLRNVPAISNR

SEQ ID NO: 363 - protein, 25 aa, Influenza virus A
  C-terminal short stem segment of Influenza A HA subtype H14
CPKYVKQGSLMLATGMRNIPGKQAK

SEQ ID NO: 364 - protein, 26 aa, Influenza virus A
  C-terminal short stem segment of Influenza A HA subtype H15
CPRYVKQSSLPLALGMKNVPEKIRTR

SEQ ID NO: 365 - protein, 25 aa, Influenza virus A
  C-terminal short stem segment of Influenza A HA subtype H16
CPKYIKSGQLKLATGLRNVPSIGER

SEQ ID NO: 366 - protein, 24 aa, Influenza virus A
  C-terminal stem segment of Influenza A HA subtype H1(no Cys)
PKYVRSAKLRMVTGLRNNPSIQSR

SEQ ID NO: 367 - protein, 23 aa, Influenza virus A
  C-terminal stem segment of Influenza A HA subtype H1(no Cys-delta 1)
KYVRSAKLRMVTGLRNNPSIQSR

SEQ ID NO: 368 - protein, 22 aa, Influenza virus A
  C-terminal stem segment of Influenza A HA subtype H1(no Cys-delta 3)
YVRSAKLRMVTGLRNNPSIQSR

SEQ ID NO: 369 - protein, 24 aa, Influenza virus A
  C-terminal stem segment of Influenza A HA subtype H2(no Cys)
PKYVKSERLVLATGLRNVPQIESR

SEQ ID NO: 370 - protein, 23 aa, Influenza virus A
  C-terminal stem segment of Influenza A HA subtype H2(no Cys-delta 1)
KYVKSERLVLATGLRNVPQIESR

SEQ ID NO: 371 - protein, 22 aa, Influenza virus A
  C-terminal stem segment of Influenza A HA subtype H2(no Cys-delta 3)
YVKSERLVLATGLRNVPQIESR

SEQ ID NO: 372 - protein, 24 aa, Influenza virus A
  C-terminal stem segment of Influenza A HA subtype H3(no Cys)
PKYVKQNTLKLATGMRNVPEKQTR

SEQ ID NO: 373 - protein, 23 aa, Influenza virus A
  C-terminal stem segment of Influenza A HA subtype H3(no Cys-delta 1)
KYVKQNTLKLATGMRNVPEKQTR

SEQ ID NO: 374 - protein, 22 aa, Influenza virus A
  C-terminal stem segment of Influenza A HA subtype H3(no Cys-delta 3)
YVKQNTLKLATGMRNVPEKQTR

SEQ ID NO: 375 - protein, 24 aa, Influenza virus A
  C-terminal stem segment of Influenza A HA subtype H4(no Cys)
PRYVKQGSLKLATGMRNIPEKASR

SEQ ID NO: 376 - protein, 23 aa, Influenza virus A
  C-terminal stem segment of Influenza A HA subtype H4(no Cys-delta 1)
RYVKQGSLKLATGMRNIPEKASR

SEQ ID NO: 377 - protein, 22 aa, Influenza virus A
  C-terminal stem segment of Influenza A HA subtype H4(no Cys-delta 3)
YVKQGSLKLATGMRNIPEKASR

SEQ ID NO: 378 - protein, 24 aa, Influenza virus A
  C-terminal stem segment of Influenza A HA subtype H5(no Cys)
PKYVKSDRLVLATGLRNVPQRKKR

SEQ ID NO: 379 - protein, 23 aa, Influenza virus A
  C-terminal stem segment of Influenza A HA subtype H5(no Cys-delta 1)
KYVKSDRLVLATGLRNVPQRKKR

SEQ ID NO: 380 - protein, 22 aa, Influenza virus A
  C-terminal stem segment of Influenza A HA subtype H5(no Cys-delta 3)
YVKSDRLVLATGLRNVPQRKKR

SEQ ID NO: 381 - protein, 24 aa, Influenza virus A
  C-terminal stem segment of Influenza A HA subtype H6(no Cys)
PKYVKSESLRLATGLRNVPQIETR

SEQ ID NO: 382 - protein, 23 aa, Influenza virus A
  C-terminal stem segment of Influenza A HA subtype H6(no Cys-delta 1)
KYVKSESLRLATGLRNVPQIETR

SEQ ID NO: 383 - protein, 22 aa, Influenza virus A
  C-terminal stem segment of Influenza A HA subtype H6(no Cys-delta 3)
YVKSESLRLATGLRNVPQIETR

SEQ ID NO: 384 - protein, 28 aa, Influenza virus A
  C-terminal stem segment of Influenza A HA subtype H7(no Cys)
PRYVKQESLLLATGMKNVPEPSKKRKKR

SEQ ID NO: 385 - protein, 27 aa, Influenza virus A
  C-terminal stem segment of Influenza A HA subtype H7(no Cys-delta 1)
RYVKQESLLLATGMKNVPEPSKKRKKR

SEQ ID NO: 386 - protein, 26 aa, Influenza virus A
  C-terminal stem segment of Influenza A HA subtype H7(no Cys-delta 3)
YVKQESLLLATGMKNVPEPSKKRKKR

SEQ ID NO: 387 - protein, 24 aa, Influenza virus A
  C-terminal stem segment of Influenza A HA subtype H8(no Cys)
PKYVKKASLRLAVGLRNTPSVEPR

SEQ ID NO: 388 - protein, 23 aa, Influenza virus A
  C-terminal stem segment of Influenza A HA subtype H8(no Cys-delta 1)
KYVKKASLRLAVGLRNTPSVEPR

SEQ ID NO: 389 - protein, 22 aa, Influenza virus A
  C-terminal stem segment of Influenza A HA subtype H8(no Cys-delta 3)
YVKKASLRLAVGLRNTPSVEPR

SEQ ID NO: 390 - protein, 24 aa, Influenza virus A
  C-terminal stem segment of Influenza A HA subtype H9(no Cys)
PKYVGVKSLKLPVGLRNVPAVSSR

SEQ ID NO: 391 - protein, 23 aa, Influenza virus A
  C-terminal stem segment of Influenza A HA subtype H9(no Cys-delta 1)
KYVGVKSLKLPVGLRNVPAVSSR

SEQ ID NO: 392 - protein, 22 aa, Influenza virus A
  C-terminal stem segment of Influenza A HA subtype H9(no Cys-delta 3)
YVGVKSLKLPVGLRNVPAVSSR

SEQ ID NO: 393 - protein, 25 aa, Influenza virus A
  C-terminal stem segment of Influenza A HA subtype H10(no Cys)
PKYVNQRSLLLATGMRNVPEVVQGR

SEQ ID NO: 394 - protein, 24 aa, Influenza virus A
  C-terminal stem segment of Influenza A HA subtype H10(no Cys-delta 1)
KYVNQRSLLLATGMRNVPEVVQGR

SEQ ID NO: 395 - protein, 23 aa, Influenza virus A
  C-terminal stem segment of Influenza A HA subtype H10(no Cys-delta 3)
YVNQRSLLLATGMRNVPEVVQGR

SEQ ID NO: 396 - protein, 24 aa, Influenza virus A
  C-terminal stem segment of Influenza A HA subtype H11(no Cys)
PKYVNVKSLKLATGPRNVPAIASR

SEQ ID NO: 397 - protein, 23 aa, Influenza virus A
  C-terminal stem segment of Influenza A HA subtype H11(no Cys-delta 1)
KYVNVKSLKLATGPRNVPAIASR

SEQ ID NO: 398 - protein, 22 aa, Influenza virus A
  C-terminal stem segment of Influenza A HA subtype H11(no Cys-delta 3)
YVNVKSLKLATGPRNVPAIASR

SEQ ID NO: 399 - protein, 24 aa, Influenza virus A
  C-terminal stem segment of Influenza A HA subtype H12(no Cys)
PKYIPSGSLKLAIGLRNVPQVQDR

SEQ ID NO: 400 - protein, 23 aa, Influenza virus A
  C-terminal stem segment of Influenza A HA subtype H12(no Cys-delta 1)
KYIPSGSLKLAIGLRNVPQVQDR

SEQ ID NO: 401 - protein, 22 aa, Influenza virus A
  C-terminal stem segment of Influenza A HA subtype H12(no Cys-delta 3)
YIPSGSLKLAIGLRNVPQVQDR

SEQ ID NO: 402 - protein, 24 aa, Influenza virus A
  C-terminal stem segment of Influenza A HA subtype H13(no Cys)
PKYIKSGQLKLATGLRNVPAISNR

SEQ ID NO: 403 - protein, 23 aa, Influenza virus A
  C-terminal stem segment of Influenza A HA subtype H13(no Cys-delta 1)
KYIKSGQLKLATGLRNVPAISNR

SEQ ID NO: 404 - protein, 22 aa, Influenza virus A
  C-terminal stem segment of Influenza A HA subtype H13(no Cys-delta 3)
YIKSGQLKLATGLRNVPAISNR

SEQ ID NO: 405 - protein, 24 aa, Influenza virus A
  C-terminal stem segment of Influenza A HA subtype H14(no Cys)
PKYVKQGSLMLATGMRNIPGKQAK

SEQ ID NO: 406 - protein, 23 aa, Influenza virus A
  C-terminal stem segment of Influenza A HA subtype H14(no Cys-delta 1)
KYVKQGSLMLATGMRNIPGKQAK

SEQ ID NO: 407 - protein, 22 aa, Influenza virus A
  C-terminal stem segment of Influenza A HA subtype H14(no Cys-delta 3)
YVKQGSLMLATGMRNIPGKQAK

SEQ ID NO: 408 - protein, 25 aa, Influenza virus A
  C-terminal stem segment of Influenza A HA subtype H15(no Cys)
PRYVKQSSLPLALGMKNVPEKIRTR

SEQ ID NO: 409 - protein, 24 aa, Influenza virus A
  C-terminal stem segment of Influenza A HA subtype H15(no Cys-delta 1)
RYVKQSSLPLALGMKNVPEKIRTR

SEQ ID NO: 410 - protein, 23 aa, Influenza virus A
  C-terminal stem segment of Influenza A HA subtype H15(no Cys-delta 3)
YVKQSSLPLALGMKNVPEKIRTR

SEQ ID NO: 411 - protein, 24 aa, Influenza virus A
  C-terminal stem segment of Influenza A HA subtype H16(no Cys)
PKYIKSGQLKLATGLRNVPSIGER

SEQ ID NO: 412 - protein, 23 aa, Influenza virus A
  C-terminal stem segment of Influenza A HA subtype H16(no Cys-delta 1)
KYIKSGQLKLATGLRNVPSIGER

SEQ ID NO: 413 - protein, 22 aa, Influenza virus A
  C-terminal stem segment of Influenza A HA subtype H16(no Cys-delta 3)
YIKSGQLKLATGLRNVPSIGER

SEQ ID NO: 414 - protein, 90 aa, Influenza virus A
  N-termianl long stem domain segment of Influenza A HA subtype H1
DTICIGYHANNSTDTVDTVLEKNVTVTHSVNLLEDSHNGKLCRLKGIAPLQLGKCNIAGWLLGNPECDPLLPVRSWSYIVETPNSENGIC

SEQ ID NO: 415 - protein, 90 aa, Influenza virus A
  N-termianl long stem domain segment of Influenza A HA subtype H2
DQICIGYHSNNSTEKVDTILERNVTVTHAQNILEKTHNGKLCKLNGIPPLELGDCSIAGWLLGNPECDRLLTVPEWSYIMEKENPRNGLC

SEQ ID NO: 416 - protein, 97 aa, Influenza virus A; identical to SEQ ID NO: 310
  N-termianl long stem domain segment of Influenza A HA subtype H3

SEQ ID NO: 417 - protein, 93 aa, Influenza virus A
  N-termianl long stem domain segment of Influenza A HA subtype H4
QNYTGNPVICMGHHAVANGTMVKTLADDQVEVVTAQELVESQNLPELCPSPLRLVDGQTCDIINGALGSPGCDHLNGAEWDVFIERPNAVDTC

SEQ ID NO: 418 - protein, 90 aa, Influenza virus A
  N-termianl long stem domain segment of Influenza A HA subtype H5
DQICIGYHANKSTKQVDTIMEKNVTVTHAQDILERTHNGKLCSLNGVKPLILRDCSVAGWLLGNPMCDEFLNLPEWLYIVEKDNPINSLC

SEQ ID NO: 419 - protein, 90 aa, Influenza virus A
  N-termianl long stem domain segment of Influenza A HA subtype H6
DKICIGYHANNSTTQIDTILEKNVTVTHSVELLENQKEERFCKILKKAPLDLKGCTIEGWILGNPQCDLLLGDQSWSYIVERPTAQNGIC

SEQ ID NO: 420 - protein, 87 aa, Influenza virus A
  N-termianl long stem domain segment of Influenza A HA subtype H7
DKICLGHHAVSNGTKVNTLTERGVEVVNATETVERTNIPKICSKGKRTTDLGQCGLLGTITGPPQCDQFLEFSADLIIERREGNDVC

SEQ ID NO: 421 - protein, 90 aa, Influenza virus A
  N-termianl long stem domain segment of Influenza A HA subtype H8
DRICIGYQSNNSTDTVNTLIEQNVPVTQTMELVETEKHPAYCNTDLGAPLELRDCKIEAVIYGNPKCDIHLKDQGWSYIVERPSAPEGMC

SEQ ID NO: 422 - protein, 90 aa, Influenza virus A
  N-termianl long stem domain segment of Influenza A HA subtype H9
DKICIGYQSTNSTETVDTLTESNVPVTHTKELLHTEHNGMLCATDLGHPLILDTCTIEGLIYGNPSCDILLGGKEWSYIVERSSAVNGMC

SEQ ID NO: 423 - protein, 88 aa, Influenza virus A
  N-termianl long stem domain segment of Influenza A HA subtype H10
LDRICLGHHAVANGTIVKTLTNEQEEVTNATETVESTNLNKLCMKGRSYKDLGNCHPVGMLIGTPVCDPHLTGTWDTLIERENAIAHC

SEQ ID NO: 424 - protein, 90 aa, Influenza virus A
  N-termianl long stem domain segment of Influenza A HA subtype H11
DEICIGYLSNNSTDKVDTIIENNVTVTSSVELVETEHTGSFCSINGKQPISLGDCSFAGWILGNPMCDELIGKTSWSYIVEKPNPTNGIC

SEQ ID NO: 425 - protein, 90 aa, Influenza virus A
  N-termianl long stem domain segment of Influenza A HA subtype H12
DKICIGYQTNNSTETVNTLSEQNVPVTQVEELVHRGIDPILCGTELGSPLVLDDCSLEGLILGNPKCDLYLNGREWSYIVERPKEMEGVC

SEQ ID NO: 426 - protein, 90 aa, Influenza virus A
  N-termianl long stem domain segment of Influenza A HA subtype H13
DRICVGYLSTNSSERVDTLLENGVPVTSSIDLIETNHTGTYCSLNGVSPVHLGDCSFEGWIVGNPACTSNFGIREWSYLIEDPAAPHGLC

SEQ ID NO: 427 - protein, 96 aa, Influenza virus A
  N-termianl long stem domain segment of Influenza A HA subtype H14
QITNGTTGNPIICLGHHAVENGTSVKTLTDNHVEVVSAKELVETNHTDELCPSPLKLVDGQDCHLINGALGSPGCDRLQDTTWDVFIERPTAVDTC

SEQ ID NO: 428 - protein, 87 aa, Influenza virus A
  N-termianl long stem domain segment of Influenza A HA subtype H15
DKICLGHHAVANGTKVNTLTERGVEVVNATETVEITGIDKVCTKGKKAVDLGSCGILGTIIGPPQCDLHLEFKADLIIERRNSSDIC

SEQ ID NO: 429 - protein, 90 aa, Influenza virus A
  N-termianl long stem domain segment of Influenza A HA subtype H16
DKICIGYLSNNSSDTVDTLTENGVPVTSSVDLVETNHTGTYCSLNGISPIHLGDCSFEGWIVGNPSCATNINIREWSYLIEDPNAPNKFC

SEQ ID NO: 430 - protein, 78 aa, Influenza virus A
  C-termianl long stem domain segment of Influenza A HA subtype H1
APMYAFALSRGFGSGIITSNASMHECNTKCQTPLGAINSSLPYQNIHPVTIGECPKYVRSAKLRMVTGLRNNPSIQSR

SEQ ID NO: 431 - protein, 78 aa, Influenza virus A
  C-termianl long stem domain segment of Influenza A HA subtype H2
APEYGFRISKRGSSGIMKTEGTLENCETKCQTPLGAINTTLPFHNVHPLTIGECPKYVKSERLVLATGLRNVPQIESR

SEQ ID NO: 432 - protein, 77 aa, Influenza virus A
  C-termianl long stem domain segment of Influenza A HA subtype H3
APRGYFKMRTGKSSIMSSDAPIDTCISECITPNGSIPNDKPFQNVNKITYGACPKYVKQNTLKLATGMRNVPEKQTR

SEQ ID NO: 433 - protein, 78 aa, Influenza virus A
  C-termianl long stem domain segment of Influenza A HA subtype H4
APRGHYKLNNQKKSTILNTAIPIGSCVSKCHTDKGSLSTTKPFQNISRIAVGDCPRYVKQGSLKLATGMRNIPEKASR

SEQ ID NO: 434 - protein, 78 aa, Influenza virus A
  C-termianl long stem domain segment of Influenza A HA subtype H5
APRYAYKIVKKGDSAIMKSGLAYGNCDTKCQTPVGEINSSMPFHNIHPHTIGECPKYVKSDRLVLATGLRNVPQRKKR

SEQ ID NO: 435 - protein, 79 aa, Influenza virus A
  C-termianl long stem domain segment of Influenza A HA subtype H6
APWYAFRFVSTSNKGAVFKSNLPIENCDATCQTVAGVLRTNKTFQNVSPLWIGECPKYVKSESLRLATGLRNVPQIETR

SEQ ID NO: 436 - protein, 81 aa, Influenza virus A
  C-termianl long stem domain segment of Influenza A HA subtype H7
APNRASFLRGKSMGIQSDVQVDANCEGECYHSGGTITSRLPFQNINSRAVGKCPRYVKQESLLLATGMKNVPEPSKKRKKR

SEQ ID NO: 437 - protein, 79 aa, Influenza virus A
  C-termianl long stem domain segment of Influenza A HA subtype H8
APEFGYLLKGESYGRIIQNEDIPIGNCNTKCQTYAGAINSSKPFQNASRHYMGECPKYVKKASLRLAVGLRNTPSVEPR

SEQ ID NO: 438 - protein, 78 aa, Influenza virus A
  C-termianl long stem domain segment of Influenza A HA subtype H9
APWYGHVLTGESHGRILKTDLNNGNCVVQCQTEKGGLNTTLPFHNISKYAFGNCPKYVGVKSLKLPVGLRNVPAVSSR

SEQ ID NO: 439 - protein, 78 aa, Influenza virus A
  C-termianl long stem domain segment of Influenza A HA subtype H10
APSRVSKLTGRDLGIQSEALIDNSCESKCFWRGGSINTKLPFQNLSPRTVGQCPKYVNQRSLLLATGMRNVPEVVQGR

SEQ ID NO: 440 - protein, 78 aa, Influenza virus A
  C-termianl long stem domain segment of Influenza A HA subtype H11
APRYAFEIVSVGNGKLFRSELNIESCSTKCQTEIGGINTNKSFHNVHRNTIGDCPKYVNVKSLKLATGPRNVPAIASR

SEQ ID NO: 441 - protein, 78 aa, Influenza virus A
  C-termianl long stem domain segment of Influenza A HA subtype H12
APEYGHLITGKSHGRILKNNLPMGQCVTECQLNEGVMNTSKPFQNTSKHYIGKCPKYIPSGSLKLAIGLRNVPQVQDR

SEQ ID NO: 442 - protein, 78 aa, Influenza virus A
  C-termianl long stem domain segment of Influenza A HA subtype H13
APRYGYIIEEYGKGRIFQSRIRMSRCNTKCQTSVGGINTNRTFQNIDKNALGDCPKYIKSGQLKLATGLRNVPAISNR

SEQ ID NO: 443 - protein, 78 aa, Influenza virus A
  C-termianl long stem domain segment of Influenza A HA subtype H14
APRGHYKISKSTKSTVLKSDKRIGSCTSPCLTDKGSIQSDKPFQNVSRIAIGNCPKYVKQGSLMLATGMRNIPGKQAK

SEQ ID NO: 444 - protein, 88 aa, Influenza virus A
  C-termianl long stem domain segment of Influenza A HA subtype H15
APDRATFLRSNAPSGIEYNGKSLGIQSDAQIDESCEGECFYSGGTINSPLPFQNIDSRAVGKCPRYVKQSSLPLALGMKNVPEKIRTR

SEQ ID NO: 445 - protein, 78 aa, Influenza virus A
  C-termianl long stem domain segment of Influenza A HA subtype H16
APRYGYIIEKYGTGRIFQSGVRMARCNTKCQTSLGGINTNKTFQNIERNALGDCPKYIKSGQLKLATGLRNVPSIGER

SEQ ID NO: 446 - protein, 89 aa, Influenza virus A
  N-termianl long stem domain segment of Influenza A HA subtype H1(No Cys, Ala)
DTICIGYHANNSTDTVDTVLEKNVTVTHSVNLLEDSHNGKLCRLKGIAPLQLGKCNIAGWLLGNPECDPLLPVRSWSYIVETPNSENGI

SEQ ID NO: 447 - protein, 89 aa, Influenza virus A; identical to SEQ ID NO: 446
  N-termianl long stem domain segment of Influenza A HA subtype H1(No Cys, Ala - Delta 1)

SEQ ID NO: 448 - protein, 88 aa, Influenza virus A
  N-termianl long stem domain segment of Influenza A HA subtype H1(No Cys, Ala - Delta 3)
DTICIGYHANNSTDTVDTVLEKNVTVTHSVNLLEDSHNGKLCRLKGIAPLQLGKCNIAGWLLGNPECDPLLPVRSWSYIVETPNSENG

SEQ ID NO: 449 - protein, 89 aa, Influenza virus A
  N-termianl long stem domain segment of Influenza A HA subtype H2(No Cys, Ala)
DQICIGYHSNNSTEKVDTILERNVTVTHAQNILEKTHNGKLCKLNGIPPLELGDCSIAGWLLGNPECDRLLTVPEWSYIMEKENPRNGL

SEQ ID NO: 450 - protein, 89 aa, Influenza virus A; identical to SEQ ID NO: 449
  N-termianl long stem domain segment of Influenza A HA subtype H2(No Cys, Ala - Delta 1)

SEQ ID NO: 451 - protein, 88 aa, Influenza virus A
  N-termianl long stem domain segment of Influenza A HA subtype H2(No Cys, Ala - Delta 3)
DQICIGYHSNNSTEKVDTILERNVTVTHAQNILEKTHNGKLCKLNGIPPLELGDCSIAGWLLGNPECDRLLTVPEWSYIMEKENPRNG

SEQ ID NO: 452 - protein, 96 aa, Influenza virus A
  N-termianl long stem domain segment of Influenza A HA subtype H3(No Cys, Ala)
QDLPGNDNSTATLCLGHHAVPNGTLVKTITDDQIEVTNATELVQSSSTGKICNNPHRILDGIDCTLIDALLGDPHCDVFQNETWDLFVERSKAFSN

SEQ ID NO: 453 - protein, 96 aa, Influenza virus A; identical to SEQ ID NO: 452
  N-termianl long stem domain segment of Influenza A HA subtype H3(No Cys, Ala - Delta 1)

SEQ ID NO: 454 - protein, 95 aa, Influenza virus A
  N-termianl long stem domain segment of Influenza A HA subtype H3(No Cys, Ala - Delta 3)
QDLPGNDNSTATLCLGHHAVPNGTLVKTITDDQIEVTNATELVQSSSTGKICNNPHRILDGIDCTLIDALLGDPHCDVFQNETWDLFVERSKAFS

SEQ ID NO: 455 - protein, 92 aa, Influenza virus A
  N-termianl long stem domain segment of Influenza A HA subtype H4(No Cys, Ala)
QNYTGNPVICMGHHAVANGTMVKTLADDQVEVVTAQELVESQNLPELCPSPLRLVDGQTCDIINGALGSPGCDHLNGAEWDVFIERPNAVDT

SEQ ID NO: 456 - protein, 92 aa, Influenza virus A; identical to SEQ ID NO: 455
  N-termianl long stem domain segment of Influenza A HA subtype H4(No Cys, Ala - Delta 1)

SEQ ID NO: 457 - protein, 91 aa, Influenza virus A
  N-termianl long stem domain segment of Influenza A HA subtype H4(No Cys, Ala - Delta 3)
QNYTGNPVICMGHHAVANGTMVKTLADDQVEVVTAQELVESQNLPELCPSPLRLVDGQTCDIINGALGSPGCDHLNGAEWDVFIERPNAVD

SEQ ID NO: 458 - protein, 89 aa, Influenza virus A
  N-termianl long stem domain segment of Influenza A HA subtype H5(No Cys, Ala)
DQICIGYHANKSTKQVDTIMEKNVTVTHAQDILERTHNGKLCSLNGVKPLILRDCSVAGWLLGNPMCDEFLNLPEWLYIVEKDNPINSL

SEQ ID NO: 459 - protein, 89 aa, Influenza virus A; identical to SEQ ID NO: 458
  N-termianl long stem domain segment of Influenza A HA subtype H5(No Cys, Ala - Delta 1)

SEQ ID NO: 460 - protein, 88 aa, Influenza virus A
  N-termianl long stem domain segment of Influenza A HA subtype H5(No Cys, Ala - Delta 3)
DQICIGYHANKSTKQVDTIMEKNVTVTHAQDILERTHNGKLCSLNGVKPLILRDCSVAGWLLGNPMCDEFLNLPEWLYIVEKDNPINS

SEQ ID NO: 461 - protein, 89 aa, Influenza virus A
  N-termianl long stem domain segment of Influenza A HA subtype H6(No Cys, Ala)
DKICIGYHANNSTTQIDTILEKNVTVTHSVELLENQKEERFCKILKKAPLDLKGCTIEGWILGNPQCDLLLGDQSWSYIVERPTAQNGI

SEQ ID NO: 462 - protein, 89 aa, Influenza virus A; identical to SEQ ID NO: 461
  N-termianl long stem domain segment of Influenza A HA subtype H6(No Cys, Ala - Delta 1)

SEQ ID NO: 463 - protein, 88 aa, Influenza virus A
  N-termianl long stem domain segment of Influenza A HA subtype H6(No Cys, Ala - Delta 3)
DKICIGYHANNSTTQIDTILEKNVTVTHSVELLENQKEERFCKILKKAPLDLKGCTIEGWILGNPQCDLLLGDQSWSYIVERPTAQNG

SEQ ID NO: 464 - protein, 86 aa, Influenza virus A
  N-termianl long stem domain segment of Influenza A HA subtype H7(No Cys, Ala)
DKICLGHHAVSNGTKVNTLTERGVEVVNATETVERTNIPKICSKGKRTTDLGQCGLLGTITGPPQCDQFLEFSADLIIERREGNDV

SEQ ID NO: 465 - protein, 86 aa, Influenza virus A; identical to SEQ ID NO: 464
  N-termianl long stem domain segment of Influenza A HA subtype H7(No Cys, Ala - Delta 1)

SEQ ID NO: 466 - protein, 85 aa, Influenza virus A
  N-termianl long stem domain segment of Influenza A HA subtype H7(No Cys, Ala - Delta 3)
DKICLGHHAVSNGTKVNTLTERGVEVVNATETVERTNIPKICSKGKRTTDLGQCGLLGTITGPPQCDQFLEFSADLIIERREGND

SEQ ID NO: 467 - protein, 89 aa, Influenza virus A
  N-termianl long stem domain segment of Influenza A HA subtype H8(No Cys, Ala)
DRICIGYQSNNSTDTVNTLIEQNVPVTQTMELVETEKHPAYCNTDLGAPLELRDCKIEAVIYGNPKCDIHLKDQGWSYIVERPSAPEGM

SEQ ID NO: 468 - protein, 89 aa, Influenza virus A; identical to SEQ ID NO: 467
  N-termianl long stem domain segment of Influenza A HA subtype H8(No Cys, Ala - Delta 1)

SEQ ID NO: 469 - protein, 88 aa, Influenza virus A
  N-termianl long stem domain segment of Influenza A HA subtype H8(No Cys, Ala - Delta 3)
DRICIGYQSNNSTDTVNTLIEQNVPVTQTMELVETEKHPAYCNTDLGAPLELRDCKIEAVIYGNPKCDIHLKDQGWSYIVERPSAPEG

SEQ ID NO: 470 - protein, 89 aa, Influenza virus A
  N-termianl long stem domain segment of Influenza A HA subtype H9(No Cys, Ala)
DKICIGYQSTNSTETVDTLTESNVPVTHTKELLHTEHNGMLCATDLGHPLILDTCTIEGLIYGNPSCDILLGGKEWSYIVERSSAVNGM

SEQ ID NO: 471 - protein, 89 aa, Influenza virus A; identical to SEQ ID NO: 470
  N-termianl long stem domain segment of Influenza A HA subtype H9(No Cys, Ala - Delta 1)

SEQ ID NO: 472 - protein, 88 aa, Influenza virus A
  N-termianl long stem domain segment of Influenza A HA subtype H9(No Cys, Ala - Delta 3)
DKICIGYQSTNSTETVDTLTESNVPVTHTKELLHTEHNGMLCATDLGHPLILDTCTIEGLIYGNPSCDILLGGKEWSYIVERSSAVNG

SEQ ID NO: 473 - protein, 87 aa, Influenza virus A
  N-termianl long stem domain segment of Influenza A HA subtype H10(No Cys, Ala)
LDRICLGHHAVANGTIVKTLTNEQEEVTNATETVESTNLNKLCMKGRSYKDLGNCHPVGMLIGTPVCDPHLTGTWDTLIERENAIAH

SEQ ID NO: 474 - protein, 87 aa, Influenza virus A; identical to SEQ ID NO: 473
  N-termianl long stem domain segment of Influenza A HA subtype H10(No Cys, Ala - Delta 1)

SEQ ID NO: 475 - protein, 86 aa, Influenza virus A
  N-termianl long stem domain segment of Influenza A HA subtype H10(No Cys, Ala - Delta 3)
LDRICLGHHAVANGTIVKTLTNEQEEVTNATETVESTNLNKLCMKGRSYKDLGNCHPVGMLIGTPVCDPHLTGTWDTLIERENAIA

SEQ ID NO: 476 - protein, 89 aa, Influenza virus A
  N-termianl long stem domain segment of Influenza A HA subtype H11(No Cys, Ala)
DEICIGYLSNNSTDKVDTIIENNVTVTSSVELVETEHTGSFCSINGKQPISLGDCSFAGWILGNPMCDELIGKTSWSYIVEKPNPTNGI

SEQ ID NO: 477 - protein, 89 aa, Influenza virus A; identical to SEQ ID NO: 476
  N-termianl long stem domain segment of Influenza A HA subtype H11(No Cys, Ala - Delta 1)

SEQ ID NO: 478 - protein, 88 aa, Influenza virus A
  N-termianl long stem domain segment of Influenza A HA subtype H11(No Cys, Ala - Delta 3)
DEICIGYLSNNSTDKVDTIIENNVTVTSSVELVETEHTGSFCSINGKQPISLGDCSFAGWILGNPMCDELIGKTSWSYIVEKPNPTNG

SEQ ID NO: 479 - protein, 89 aa, Influenza virus A
  N-termianl long stem domain segment of Influenza A HA subtype H12(No Cys, Ala)
DKICIGYQTNNSTETVNTLSEQNVPVTQVEELVHRGIDPILCGTELGSPLVLDDCSLEGLILGNPKCDLYLNGREWSYIVERPKEMEGV

SEQ ID NO: 480 - protein, 89 aa, Influenza virus A; identical to SEQ ID NO: 479
  N-termianl long stem domain segment of Influenza A HA subtype H12(No Cys, Ala - Delta 1)

SEQ ID NO: 481 - protein, 88 aa, Influenza virus A
  N-termianl long stem domain segment of Influenza A HA subtype H12(No Cys, Ala - Delta 3)
DKICIGYQTNNSTETVNTLSEQNVPVTQVEELVHRGIDPILCGTELGSPLVLDDCSLEGLILGNPKCDLYLNGREWSYIVERPKEMEG

SEQ ID NO: 482 - protein, 89 aa, Influenza virus A
  N-termianl long stem domain segment of Influenza A HA subtype H13(No Cys, Ala)
DRICVGYLSTNSSERVDTLLENGVPVTSSIDLIETNHTGTYCSLNGVSPVHLGDCSFEGWIVGNPACTSNFGIREWSYLIEDPAAPHGL

SEQ ID NO: 483 - protein, 89 aa, Influenza virus A; identical to SEQ ID NO: 482
  N-termianl long stem domain segment of Influenza A HA subtype H13(No Cys, Ala - Delta 1)

SEQ ID NO: 484 - protein, 88 aa, Influenza virus A
  N-termianl long stem domain segment of Influenza A HA subtype H13(No Cys, Ala - Delta 3)
DRICVGYLSTNSSERVDTLLENGVPVTSSIDLIETNHTGTYCSLNGVSPVHLGDCSFEGWIVGNPACTSNFGIREWSYLIEDPAAPHG

SEQ ID NO: 485 - protein, 95 aa, Influenza virus A
  N-termianl long stem domain segment of Influenza A HA subtype H14(No Cys, Ala)
QITNGTTGNPIICLGHHAVENGTSVKTLTDNHVEVVSAKELVETNHTDELCPSPLKLVDGQDCHLINGALGSPGCDRLQDTTWDVFIERPTAVDT

SEQ ID NO: 486 - protein, 95 aa, Influenza virus A; identical to SEQ ID NO: 485
  N-termianl long stem domain segment of Influenza A HA subtype H14(No Cys, Ala - Delta 1)

SEQ ID NO: 487 - protein, 94 aa, Influenza virus A
  N-termianl long stem domain segment of Influenza A HA subtype H14(No Cys, Ala - Delta 3)
QITNGTTGNPIICLGHHAVENGTSVKTLTDNHVEVVSAKELVETNHTDELCPSPLKLVDGQDCHLINGALGSPGCDRLQDTTWDVFIERPTAVD

SEQ ID NO: 488 - protein, 86 aa, Influenza virus A
  N-termianl long stem domain segment of Influenza A HA subtype H15(No Cys, Ala)
DKICLGHHAVANGTKVNTLTERGVEVVNATETVEITGIDKVCTKGKKAVDLGSCGILGTIIGPPQCDLHLEFKADLIIERRNSSDI

SEQ ID NO: 489 - protein, 86 aa, Influenza virus A; identical to SEQ ID NO: 488
  N-termianl long stem domain segment of Influenza A HA subtype H15(No Cys, Ala - Delta 1)

SEQ ID NO: 490 - protein, 85 aa, Influenza virus A
  N-termianl long stem domain segment of Influenza A HA subtype H15(No Cys, Ala - Delta 3)
DKICLGHHAVANGTKVNTLTERGVEVVNATETVEITGIDKVCTKGKKAVDLGSCGILGTIIGPPQCDLHLEFKADLIIERRNSSD

SEQ ID NO: 491 - protein, 89 aa, Influenza virus A
  N-termianl long stem domain segment of Influenza A HA subtype H16(No Cys, Ala)
DKICIGYLSNNSSDTVDTLTENGVPVTSSVDLVETNHTGTYCSLNGISPIHLGDCSFEGWIVGNPSCATNINIREWSYLIEDPNAPNKF

SEQ ID NO: 492 - protein, 89 aa, Influenza virus A; identical to SEQ ID NO: 491
  N-termianl long stem domain segment of Influenza A HA subtype H16(No Cys, Ala - Delta 1)

SEQ ID NO: 493 - protein, 88 aa, Influenza virus A
  N-termianl long stem domain segment of Influenza A HA subtype H16(No Cys, Ala - Delta 3)
DKICIGYLSNNSSDTVDTLTENGVPVTSSVDLVETNHTGTYCSLNGISPIHLGDCSFEGWIVGNPSCATNINIREWSYLIEDPNAPNK

SEQ ID NO: 494 - protein, 77 aa, Influenza virus A
  C-termianl long stem domain segment of Influenza A HA subtype H1(No Cys, Ala)
PMYAFALSRGFGSGIITSNASMHECNTKCQTPLGAINSSLPYQNIHPVTIGECPKYVRSAKLRMVTGLRNNPSIQSR

SEQ ID NO: 495 - protein, 76 aa, Influenza virus A
  C-termianl long stem domain segment of Influenza A HA subtype H1(No Cys, Ala - Delta 1)
MYAFALSRGFGSGIITSNASMHECNTKCQTPLGAINSSLPYQNIHPVTIGECPKYVRSAKLRMVTGLRNNPSIQSR

SEQ ID NO: 496 - protein, 75 aa, Influenza virus A
  C-termianl long stem domain segment of Influenza A HA subtype H1(No Cys, Ala - Delta 3)
YAFALSRGFGSGIITSNASMHECNTKCQTPLGAINSSLPYQNIHPVTIGECPKYVRSAKLRMVTGLRNNPSIQSR

SEQ ID NO: 497 - protein, 77 aa, Influenza virus A
  C-termianl long stem domain segment of Influenza A HA subtype H2(No Cys, Ala)
PEYGFRISKRGSSGIMKTEGTLENCETKCQTPLGAINTTLPFHNVHPLTIGECPKYVKSERLVLATGLRNVPQIESR

SEQ ID NO: 498 - protein, 76 aa, Influenza virus A
  C-termianl long stem domain segment of Influenza A HA subtype H2(No Cys, Ala - Delta 1)
EYGFRISKRGSSGIMKTEGTLENCETKCQTPLGAINTTLPFHNVHPLTIGECPKYVKSERLVLATGLRNVPQIESR

SEQ ID NO: 499 - protein, 75 aa, Influenza virus A
  C-termianl long stem domain segment of Influenza A HA subtype H2(No Cys, Ala - Delta 3)
YGFRISKRGSSGIMKTEGTLENCETKCQTPLGAINTTLPFHNVHPLTIGECPKYVKSERLVLATGLRNVPQIESR

SEQ ID NO: 500 - protein, 76 aa, Influenza virus A
  C-termianl long stem domain segment of Influenza A HA subtype H3(No Cys, Ala)
PRGYFKMRTGKSSIMSSDAPIDTCISECITPNGSIPNDKPFQNVNKITYGACPKYVKQNTLKLATGMRNVPEKQTR

SEQ ID NO: 501 - protein, 75 aa, Influenza virus A
  C-termianl long stem domain segment of Influenza A HA subtype H3(No Cys, Ala - Delta 1)
RGYFKMRTGKSSIMSSDAPIDTCISECITPNGSIPNDKPFQNVNKITYGACPKYVKQNTLKLATGMRNVPEKQTR

SEQ ID NO: 502 - protein, 74 aa, Influenza virus A
  C-termianl long stem domain segment of Influenza A HA subtype H3(No Cys, Ala - Delta 3)
GYFKMRTGKSSIMSSDAPIDTCISECITPNGSIPNDKPFQNVNKITYGACPKYVKQNTLKLATGMRNVPEKQTR

SEQ ID NO: 503 - protein, 77 aa, Influenza virus A
  C-termianl long stem domain segment of Influenza A HA subtype H4(No Cys, Ala)
PRGHYKLNNQKKSTILNTAIPIGSCVSKCHTDKGSLSTTKPFQNISRIAVGDCPRYVKQGSLKLATGMRNIPEKASR

SEQ ID NO: 504 - protein, 76 aa, Influenza virus A
  C-termianl long stem domain segment of Influenza A HA subtype H4(No Cys, Ala - Delta 1)
RGHYKLNNQKKSTILNTAIPIGSCVSKCHTDKGSLSTTKPFQNISRIAVGDCPRYVKQGSLKLATGMRNIPEKASR

SEQ ID NO: 505 - protein, 75 aa, Influenza virus A
  C-termianl long stem domain segment of Influenza A HA subtype H4(No Cys, Ala - Delta 3)
GHYKLNNQKKSTILNTAIPIGSCVSKCHTDKGSLSTTKPFQNISRIAVGDCPRYVKQGSLKLATGMRNIPEKASR

SEQ ID NO: 506 - protein, 77 aa, Influenza virus A
  C-termianl long stem domain segment of Influenza A HA subtype H5(No Cys, Ala)
PRYAYKIVKKGDSAIMKSGLAYGNCDTKCQTPVGEINSSMPFHNIHPHTIGECPKYVKSDRLVLATGLRNVPQRKKR

SEQ ID NO: 507 - protein, 76 aa, Influenza virus A
  C-termianl long stem domain segment of Influenza A HA subtype H5(No Cys, Ala - Delta 1)
RYAYKIVKKGDSAIMKSGLAYGNCDTKCQTPVGEINSSMPFHNIHPHTIGECPKYVKSDRLVLATGLRNVPQRKKR

SEQ ID NO: 508 - protein, 75 aa, Influenza virus A
  C-termianl long stem domain segment of Influenza A HA subtype H5(No Cys, Ala - Delta 3)
YAYKIVKKGDSAIMKSGLAYGNCDTKCQTPVGEINSSMPFHNIHPHTIGECPKYVKSDRLVLATGLRNVPQRKKR

SEQ ID NO: 509 - protein, 78 aa, Influenza virus A
  C-termianl long stem domain segment of Influenza A HA subtype H6(No Cys, Ala)
PWYAFRFVSTSNKGAVFKSNLPIENCDATCQTVAGVLRTNKTFQNVSPLWIGECPKYVKSESLRLATGLRNVPQIETR

SEQ ID NO: 510 - protein, 77 aa, Influenza virus A
  C-termianl long stem domain segment of Influenza A HA subtype H6(No Cys, Ala - Delta 1)
WYAFRFVSTSNKGAVFKSNLPIENCDATCQTVAGVLRTNKTFQNVSPLWIGECPKYVKSESLRLATGLRNVPQIETR

SEQ ID NO: 511 - protein, 76 aa, Influenza virus A
  C-termianl long stem domain segment of Influenza A HA subtype H6(No Cys, Ala - Delta 3)
YAFRFVSTSNKGAVFKSNLPIENCDATCQTVAGVLRTNKTFQNVSPLWIGECPKYVKSESLRLATGLRNVPQIETR

SEQ ID NO: 512 - protein, 80 aa, Influenza virus A
  C-termianl long stem domain segment of Influenza A HA subtype H7(No Cys, Ala)
PNRASFLRGKSMGIQSDVQVDANCEGECYHSGGTITSRLPFQNINSRAVGKCPRYVKQESLLLATGMKNVPEPSKKRKKR

SEQ ID NO: 513 - protein, 79 aa, Influenza virus A
  C-termianl long stem domain segment of Influenza A HA subtype H7(No Cys, Ala - Delta 1)
NRASFLRGKSMGIQSDVQVDANCEGECYHSGGTITSRLPFQNINSRAVGKCPRYVKQESLLLATGMKNVPEPSKKRKKR

SEQ ID NO: 514 - protein, 78 aa, Influenza virus A
  C-termianl long stem domain segment of Influenza A HA subtype H7(No Cys, Ala - Delta 3)
RASFLRGKSMGIQSDVQVDANCEGECYHSGGTITSRLPFQNINSRAVGKCPRYVKQESLLLATGMKNVPEPSKKRKKR

SEQ ID NO: 515 - protein, 78 aa, Influenza virus A
  C-termianl long stem domain segment of Influenza A HA subtype H8(No Cys, Ala)
PEFGYLLKGESYGRIIQNEDIPIGNCNTKCQTYAGAINSSKPFQNASRHYMGECPKYVKKASLRLAVGLRNTPSVEPR

SEQ ID NO: 516 - protein, 77 aa, Influenza virus A
  C-termianl long stem domain segment of Influenza A HA subtype H8(No Cys, Ala - Delta 1)
EFGYLLKGESYGRIIQNEDIPIGNCNTKCQTYAGAINSSKPFQNASRHYMGECPKYVKKASLRLAVGLRNTPSVEPR

SEQ ID NO: 517 - protein, 76 aa, Influenza virus A
  C-termianl long stem domain segment of Influenza A HA subtype H8(No Cys, Ala - Delta 3)
FGYLLKGESYGRIIQNEDIPIGNCNTKCQTYAGAINSSKPFQNASRHYMGECPKYVKKASLRLAVGLRNTPSVEPR

SEQ ID NO: 518 - protein, 77 aa, Influenza virus A
  C-termianl long stem domain segment of Influenza A HA subtype H9(No Cys, Ala)
PWYGHVLTGESHGRILKTDLNNGNCVVQCQTEKGGLNTTLPFHNISKYAFGNCPKYVGVKSLKLPVGLRNVPAVSSR

SEQ ID NO: 519 - protein, 76 aa, Influenza virus A
  C-termianl long stem domain segment of Influenza A HA subtype H9(No Cys, Ala - Delta 1)
WYGHVLTGESHGRILKTDLNNGNCVVQCQTEKGGLNTTLPFHNISKYAFGNCPKYVGVKSLKLPVGLRNVPAVSSR

SEQ ID NO: 520 - protein, 75 aa, Influenza virus A
  C-termianl long stem domain segment of Influenza A HA subtype H9(No Cys, Ala - Delta 3)
YGHVLTGESHGRILKTDLNNGNCVVQCQTEKGGLNTTLPFHNISKYAFGNCPKYVGVKSLKLPVGLRNVPAVSSR

SEQ ID NO: 521 - protein, 77 aa, Influenza virus A
  C-termianl long stem domain segment of Influenza A HA subtype H10(No Cys, Ala)
PSRVSKLTGRDLGIQSEALIDNSCESKCFWRGGSINTKLPFQNLSPRTVGQCPKYVNQRSLLLATGMRNVPEVVQGR

SEQ ID NO: 522 - protein, 76 aa, Influenza virus A
  C-termianl long stem domain segment of Influenza A HA subtype H10(No Cys, Ala - Delta 1)
SRVSKLTGRDLGIQSEALIDNSCESKCFWRGGSINTKLPFQNLSPRTVGQCPKYVNQRSLLLATGMRNVPEVVQGR

SEQ ID NO: 523 - protein, 75 aa, Influenza virus A
  C-termianl long stem domain segment of Influenza A HA subtype H10(No Cys, Ala - Delta 3)
RVSKLTGRDLGIQSEALIDNSCESKCFWRGGSINTKLPFQNLSPRTVGQCPKYVNQRSLLLATGMRNVPEVVQGR

SEQ ID NO: 524 - protein, 77 aa, Influenza virus A
  C-termianl long stem domain segment of Influenza A HA subtype H11(No Cys, Ala)
PRYAFEIVSVGNGKLFRSELNIESCSTKCQTEIGGINTNKSFHNVHRNTIGDCPKYVNVKSLKLATGPRNVPAIASR

SEQ ID NO: 525 - protein, 76 aa, Influenza virus A
  C-termianl long stem domain segment of Influenza A HA subtype H11(No Cys, Ala - Delta 1)
RYAFEIVSVGNGKLFRSELNIESCSTKCQTEIGGINTNKSFHNVHRNTIGDCPKYVNVKSLKLATGPRNVPAIASR

SEQ ID NO: 526 - protein, 75 aa, Influenza virus A
  C-termianl long stem domain segment of Influenza A HA subtype H11(No Cys, Ala - Delta 3)
YAFEIVSVGNGKLFRSELNIESCSTKCQTEIGGINTNKSFHNVHRNTIGDCPKYVNVKSLKLATGPRNVPAIASR

SEQ ID NO: 527 - protein, 77 aa, Influenza virus A
  C-termianl long stem domain segment of Influenza A HA subtype H12(No Cys, Ala)
PEYGHLITGKSHGRILKNNLPMGQCVTECQLNEGVMNTSKPFQNTSKHYIGKCPKYIPSGSLKLAIGLRNVPQVQDR

SEQ ID NO: 528 - protein, 76 aa, Influenza virus A
  C-termianl long stem domain segment of Influenza A HA subtype H12(No Cys, Ala - Delta 1)
EYGHLITGKSHGRILKNNLPMGQCVTECQLNEGVMNTSKPFQNTSKHYIGKCPKYIPSGSLKLAIGLRNVPQVQDR

SEQ ID NO: 529 - protein, 75 aa, Influenza virus A
  C-termianl long stem domain segment of Influenza A HA subtype H12(No Cys, Ala - Delta 3)
YGHLITGKSHGRILKNNLPMGQCVTECQLNEGVMNTSKPFQNTSKHYIGKCPKYIPSGSLKLAIGLRNVPQVQDR

SEQ ID NO: 530 - protein, 77 aa, Influenza virus A
  C-termianl long stem domain segment of Influenza A HA subtype H13(No Cys, Ala)
PRYGYIIEEYGKGRIFQSRIRMSRCNTKCQTSVGGINTNRTFQNIDKNALGDCPKYIKSGQLKLATGLRNVPAISNR

SEQ ID NO: 531 - protein, 76 aa, Influenza virus A
  C-termianl long stem domain segment of Influenza A HA subtype H13(No Cys, Ala - Delta 1)
RYGYIIEEYGKGRIFQSRIRMSRCNTKCQTSVGGINTNRTFQNIDKNALGDCPKYIKSGQLKLATGLRNVPAISNR

SEQ ID NO: 532 - protein, 75 aa, Influenza virus A
  C-termianl long stem domain segment of Influenza A HA subtype H13(No Cys, Ala - Delta 3)
YGYIIEEYGKGRIFQSRIRMSRCNTKCQTSVGGINTNRTFQNIDKNALGDCPKYIKSGQLKLATGLRNVPAISNR

SEQ ID NO: 533 - protein, 77 aa, Influenza virus A
  C-termianl long stem domain segment of Influenza A HA subtype H14(No Cys, Ala)
PRGHYKISKSTKSTVLKSDKRIGSCTSPCLTDKGSIQSDKPFQNVSRIAIGNCPKYVKQGSLMLATGMRNIPGKQAK

SEQ ID NO: 534 - protein, 76 aa, Influenza virus A
  C-termianl long stem domain segment of Influenza A HA subtype H14(No Cys, Ala - Delta 1)
RGHYKISKSTKSTVLKSDKRIGSCTSPCLTDKGSIQSDKPFQNVSRIAIGNCPKYVKQGSLMLATGMRNIPGKQAK

SEQ ID NO: 535 - protein, 75 aa, Influenza virus A
  C-termianl long stem domain segment of Influenza A HA subtype H14(No Cys, Ala - Delta 3)
GHYKISKSTKSTVLKSDKRIGSCTSPCLTDKGSIQSDKPFQNVSRIAIGNCPKYVKQGSLMLATGMRNIPGKQAK

SEQ ID NO: 536 - protein, 87 aa, Influenza virus A
  C-termianl long stem domain segment of Influenza A HA subtype H15(No Cys, Ala)
PDRATFLRSNAPSGIEYNGKSLGIQSDAQIDESCEGECFYSGGTINSPLPFQNIDSRAVGKCPRYVKQSSLPLALGMKNVPEKIRTR

SEQ ID NO: 537 - protein, 86 aa, Influenza virus A
  C-termianl long stem domain segment of Influenza A HA subtype H15(No Cys, Ala - Delta 1)
DRATFLRSNAPSGIEYNGKSLGIQSDAQIDESCEGECFYSGGTINSPLPFQNIDSRAVGKCPRYVKQSSLPLALGMKNVPEKIRTR

SEQ ID NO: 538 - protein, 85 aa, Influenza virus A
  C-termianl long stem domain segment of Influenza A HA subtype H15(No Cys, Ala - Delta 3)
RATFLRSNAPSGIEYNGKSLGIQSDAQIDESCEGECFYSGGTINSPLPFQNIDSRAVGKCPRYVKQSSLPLALGMKNVPEKIRTR

SEQ ID NO: 539 - protein, 77 aa, Influenza virus A
  C-termianl long stem domain segment of Influenza A HA subtype H16(No Cys, Ala)
PRYGYIIEKYGTGRIFQSGVRMARCNTKCQTSLGGINTNKTFQNIERNALGDCPKYIKSGQLKLATGLRNVPSIGER

SEQ ID NO: 540 - protein, 76 aa, Influenza virus A
  C-termianl long stem domain segment of Influenza A HA subtype H16(No Cys, Ala - Delta 1)
RYGYIIEKYGTGRIFQSGVRMARCNTKCQTSLGGINTNKTFQNIERNALGDCPKYIKSGQLKLATGLRNVPSIGER

SEQ ID NO: 541 - protein, 75 aa, Influenza virus A
  C-termianl long stem domain segment of Influenza A HA subtype H16(No Cys, Ala - Delta 3)
YGYIIEKYGTGRIFQSGVRMARCNTKCQTSLGGINTNKTFQNIERNALGDCPKYIKSGQLKLATGLRNVPSIGER

SEQ ID NO: 542 - protein, 16 aa, Artificial Sequence
  linker sequence
KLNGSGIMKTEGTLEN

SEQ ID NO: 543 - protein, 5 aa, Artificial Sequence
  linker sequence
NNIDT

SEQ ID NO: 544 - protein, 5 aa, Artificial Sequence
  sequence of influenza HA polypeptide
TGLRN

SEQ ID NO: 545 - protein, 12 aa, Artificial Sequence
  sequence of influenza HA polypeptide
GITNKVNSVIEK

SEQ ID NO: 546 - protein, 5 aa, Artificial Sequence
  linker sequence
NNIDT

SEQ ID NO: 547 - protein, 5 aa, Artificial Sequence
  sequence of influenza HA polypeptide
TGMRN

SEQ ID NO: 548 - protein, 12 aa, Artificial Sequence
  sequence of influenza HA polypeptide
QINGKLNRLIEK

SEQ ID NO: 549 - protein, 12 aa, Artificial Sequence
  sequence of influenza HA polypeptide
QINGKLNRVIEK

SEQ ID NO: 550 - protein, 94 aa, Influenza virus B
  HA1 N-terminal Stem Segment of Influenza B HA construct variant Cys94-Cys143
DRICTGITSSNSPHVVKTATQGEVNVTGVIPLTTTPTKSHFANLKGTQTRGKLCPNCLNCTDLDVALGRPKCMGTIPSAKASILHEVKPVTSGC

SEQ ID NO: 551 - protein, 178 aa, Influenza virus B
  HA1 N-terminal Stem Segment of Influenza B HA construct variant Cys178-Cys272
DRICTGITSSNSPHVVKTATQGEVNVTGVIPLTTTPTKSHFANLKGTQTRGKLCPNCLNCTDLDVALGRPKCMGTIPSAKASILHEVKPVTSGCFPIMHDRTKIRQLPNLLRGYENIRLSARNVTNAETAPGGPYIVGTSGSCPNVTNGNGFFATMAWAVPKNKTATNPLTVEVPYIC

SEQ ID NO: 552 - protein, 54 aa, Influenza virus B
  HA1 N-terminal Stem Segment of Influenza B HA construct variant Cys54-Cys272
DRICTGITSSNSPHVVKTATQGEVNVTGVIPLTTTPTKSHFANLKGTQTRGKLC

SEQ ID NO: 553 - protein, 200 aa, Influenza virus B
  HA1 C-terminal Stem Segment of Influenza B HA construct variant Cys94-Cys143
CPNVTNGNGFFATMAWAVPKNKTATNPLTVEVPYICTKGEDQITVWGFHSDDETQMVKLYGDSKPQKFTSSANGVTTHYVSQIGGFPNQAEDEGLPQSGRIVVDYMVQKPGKTGTIAYQRGVLLPQKVWCASGRSKVIKGSLPLIGEADCLHEKYGGLNKSKPYYTGEHAKAIGNCPIWVKTPLKLANGTKYRPPAKLLK

SEQ ID NO: 554 - protein, 71 aa, Influenza virus B
  HA1 C-terminal Stem Segment of Influenza B HA construct variant Cys178-Cys272
CASGRSKVIKGSLPLIGEADCLHEKYGGLNKSKPYYTGEHAKAIGNCPIWVKTPLKLANGTKYRPPAKLLK

SEQ ID NO: 555 - protein, 94 aa, Influenza virus B; identical to SEQ ID NO: 550
  HA1 N-terminal Stem Segment of Influenza B HA construct variant Cys94-Cys143-Cys178-Cys272

SEQ ID NO: 556 - protein, 36 aa, Influenza virus B
  HA1 intermediate Segment of Influenza B HA construct variant Cys94-Cys143-Cys178-Cys272
CPNVTNGNGFFATMAWAVPKNKTATNPLTVEVPYIC

SEQ ID NO: 557 - protein, 71 aa, Influenza virus B; identical to SEQ ID NO: 554
  HA1 C-terminal Stem Segment of Influenza B HA construct variant Cys94-Cys143-Cys178-Cys272

SEQ ID NO: 558 - protein, 585 aa, Influenza virus B
  representative sequence of influenza virus B hemagglutinin (in Fig. 2)
MKAIIVILMVVTSNADRICTGITSSNSPHVVKTATQGEVNVTGVIPLTTTPTKSHFANLKGTETRGKLCPKCLNCTDLDVALGRPKCTGKIPSARVSILHEVRPVTSGCFPIMHDRTKIRQLPNLLRGYEHIRLSTHNVINAENAPGGPYKIGTSGSCPNITNGNGFFATMAWAVPKNDKNKTATNPLTIEVPYICTEGEDQITVWGFHSDSETQMAKLYGDSKPQKFTSSANGVTTHYVSQIGGFPNQTEDGGLPQSGRIVVDYMVQKSGKTGTITYQRGILLPQKVWCASGRSKVIKGSLPLIGEADCLHEKYGGLNKSKPYYTGEHAKAIGNCPIWVKTPLKLANGTKYRPPAKLLKERGFFGAIAGFLEGGWEGMIAGWHGYTSHGAHGVAVAADLKSTQEAINKITKNLNSLSELEVKNLQRLSGAMDELHNEILELDEKVDDLRADTISSQIELAVLLSNETFDSLNITAASLNDDGLDNHTILLYYSTAASSLAVTLMIAIFVVYMVSRDNVSCSICLGIINSEDEHLLALERKLKKMLGPSAVEIGNGCFETKHKCNQTCLDRIAAGTFDAGEFSLP

SEQ ID NO: 559 - protein, 16 aa, Artificial Sequence
  linker sequence
KLNGSGIMKTEGTLEN

SEQ ID NO: 560 - protein, 18 aa, Artificial Sequence
  influenza A HA subtype H17 signal peptides
MELIVLLILLNPYTFVLG

SEQ ID NO: 561 - protein, 42 aa, Artificial Sequence
  influenza A HA subtype H17 N-terminal stem segment
DRICIGYQANQNNQTVNTLLEQNVPVTGAQEILETNHNGKLC

SEQ ID NO: 562 - protein, 53 aa, Artificial Sequence
  influenza A HA subtype H17 C-terminal stem segment
CSTKCQTPLGALNSTLPFQNVHQQTIGNCPKYVKATSLMLATGLRNNPQMEGR

SEQ ID NO: 563 - protein, 222 aa, Artificial Sequence
  influenza A HA subtype H17 HA2 domain
GLFGAIAGFIEGGWQGMIDGWYGYHHENQEGSGYAADKEATQKAVDAITNKVNSIIDKMNSQFESNIKEFNRLELRIQHLSDRVDDALLDIWSYNTELLVLLENERTLDFHDANVKNLFEKVKAQLKDNAIDEGNGCFLLLHKCNNSCMDDIKNGTYKYMDYREESHIEKQKIDGVKLTDYSRYYIMTLYSTIASSVVLGSLIIAAFLWGCQKGSIQCKICI

SEQ ID NO: 564 - protein, 41 aa, Artificial Sequence
  N-terminal stem segment of Influenza A HA subtype H17(no Cys)
DRICIGYQANQNNQTVNTLLEQNVPVTGAQEILETNHNGKL

SEQ ID NO: 565 - protein, 52 aa, Artificial Sequence
  C-terminal stem segment of Influenza A HA subtype H17(no Cys)
STKCQTPLGALNSTLPFQNVHQQTIGNCPKYVKATSLMLATGLRNNPQMEGR

SEQ ID NO: 566 - protein, 180 aa, Artificial Sequence
  influenza A HA2 domain subtype H17 stem domain
GLFGAIAGFIEGGWQGMIDGWYGYHHENQEGSGYAADKEATQKAVDAITNKVNSIIDKMNSQFESNIKEFNRLELRIQHLSDRVDDALLDIWSYNTELLVLLENERTLDFHDANVKNLFEKVKAQLKDNAIDEGNGCFLLLHKCNNSCMDDIKNGTYKYMDYREESHIEKQKIDGVKLTD

SEQ ID NO: 567 - protein, 5 aa, Artificial Sequence
  influenza A HA2 domain subtype H17 luminal domain
YSRYY

SEQ ID NO: 568 - protein, 27 aa, Artificial Sequence
  influenza A HA2 domain subtype H17 transmembrane domain
IMTLYSTIASSVVLGSLIIAAFLWGCQ

SEQ ID NO: 569 - protein, 10 aa, Artificial Sequence
  influenza A HA2 domain subtype H17 cytoplasmic domain
KGSIQCKICI

SEQ ID NO: 570 - protein, 18 aa, Artificial Sequence
  influenza A HA subtype H17 signal peptide
MELIVLLILLNPYTFVLG

SEQ ID NO: 571 - protein, 42 aa, Artificial Sequence; identical to SEQ ID NO: 561
  influenza A HA subtype H17 N-terminal stem segment

SEQ ID NO: 572 - protein, 25 aa, Artificial Sequence
  influenza A HA subtype H17 C-terminal short stem segment
CPKYVKATSLMLATGLRNNPQMEGR

SEQ ID NO: 573 - protein, 222 aa, Artificial Sequence; identical to SEQ ID NO: 563
  influenza A HA subtype H17 HA2 domain

SEQ ID NO: 574 - protein, 41 aa, Artificial Sequence; identical to SEQ ID NO: 564
  influenza A HA subtype H17 N-terminal stem segment

SEQ ID NO: 575 - protein, 24 aa, Artificial Sequence
  influenza A HA subtype H17 C-terminal stem segment
PKYVKATSLMLATGLRNNPQMEGR

SEQ ID NO: 576 - protein, 18 aa, Artificial Sequence
  influenza A HA subtype H17 signal peptide
MELIVLLILLNPYTFVLG

SEQ ID NO: 577 - protein, 90 aa, Artificial Sequence
  influenza A HA subtype H17 N-terminal long stem segment
DRICIGYQANQNNQTVNTLLEQNVPVTGAQEILETNHNGKLCSLNGVPPLDLQSCTLAGWLLGNPNCDSLLEAEEWSYIKINESAPDDLC

SEQ ID NO: 578 - protein, 79 aa, Artificial Sequence
  influenza A HA subtype H17 C-terminal long stem segment
APEYGFYYKRKEGKGGLMKSKLPISDCSTKCQTPLGALNSTLPFQNVHQQTIGNCPKYVKATSLMLATGLRNNPQMEGR

SEQ ID NO: 579 - protein, 222 aa, Artificial Sequence; identical to SEQ ID NO: 563
  influenza A HA subtype H17 HA2 domain

SEQ ID NO: 580 - protein, 89 aa, Artificial Sequence
  influenza A HA subtype H17 N-terminal long stem segment
DRICIGYQANQNNQTVNTLLEQNVPVTGAQEILETNHNGKLCSLNGVPPLDLQSCTLAGWLLGNPNCDSLLEAEEWSYIKINESAPDDL

SEQ ID NO: 581 - protein, 78 aa, Artificial Sequence
  influenza A HA subtype H17 C-terminal long stem segment
PEYGFYYKRKEGKGGLMKSKLPISDCSTKCQTPLGALNSTLPFQNVHQQTIGNCPKYVKATSLMLATGLRNNPQMEGR

SEQ ID NO: 582 - protein, 7 aa, Artificial Sequence
  a cleavage site recognized by Tobacco Etch Virus (TEV) protease
  Variant 7: Xaa = Gly or Ser
ENLYFQX